European Patent Application EP 4 678 010 A1, published January 14, 2026. Title: Flavour composition comprising a heme protein. Applicant: Paleo B.V. The sequence listing filed with the application follows.

SEQUENCE LISTING (28 sequences)

SEQ ID NO: 1 - protein, 154 aa, Mammuthus trogontherii
  source 1..154: note = Amino acid sequence of steppe mammoth myoglobin
MGLSDGEWELVLKTWGKVEADIPGHGLEVFVRLFTGHPETLEKFDKFKHLKTEGEMKASEDLKKQGVTVLTALGGILKKKGHHQAEIQPLAHSHATKHKIPIKYLEFISDAIIHVLQSKHPAEFGADAQGAMKKALELFRNDIAAKYKELGFQG

SEQ ID NO: 2 - protein, 154 aa, Mammuthus primigenius
  source 1..154: note = Amino acid sequence of woolly mammoth myoglobin
MGLSDGEWELVLKTWGKVEADIPGHGLEVFVRLFTGHPETLEKFDKFKHLKTEGEMKASEDLKKQGVTVLTALGGILKKKGHHQAEIQPLAQSHATKHKIPIKYLEFISDAIIHVLQSKHPAEFGADAQGAMKKALELFRNDIAAKYKELGFQG

SEQ ID NO: 3 - protein, 147 aa, Thunnus orientalis
  source 1..147: note = Amino acid sequence of pig myoglobin
MADFDAVLKCWGPVEADYTTMGGLVLTRLFKEHPETQKLFPKFAGIAQADIAGNAAISAHGATVLKKLGELLKAKGSHAAILKPLANSHATKHKIPINNFKLISEVLVKVMHEKAGLDAGQQTALRNVMGIIIADLEANYKELGFSG

SEQ ID NO: 4 - protein, 154 aa, Ovies aries
  source 1..154: note = Amino acid sequence of sheep myoglobin
MGLSDGEWQLVLNAWGKVEADVAGHGQEVLIRLFTGHPETLEKFDKFKHLKTEAEMKASEDLKKHGNTVLTALGGILKKKGHHEAEVKHLAESHANKHKIPVKYLEFISDAIIHVLHAKHPSDFGADAQGAMSKALELFRNDMAAQYKVLGFQG

SEQ ID NO: 5 - protein, 154 aa, Bos taurus
  source 1..154: note = Amino acid sequence of cow myoglobin
MGLSDGEWQLVLNAWGKVEADVAGHGQEVLIRLFTGHPETLEKFDKFKHLKTEAEMKASEDLKKHGNTVLTALGGILKKKGHHEAEVKHLAESHANKHKIPVKYLEFISDAIIHVLHAKHPSDFGADAQAAMSKALELFRNDMAAQYKVLGFHG

SEQ ID NO: 6 - protein, 154 aa, Gallus gallus
  source 1..154: note = Amino acid sequence of chicken myoglobin
MGLSDQEWQQVLTIWGKVEADIAGHGHEVLMRLFHDHPETLDRFDKFKGLKTPDQMKGSEDLKKHGATVLTQLGKILKQKGNHESELKPLAQTHATKHKIPVKYLEFISEVIIKVIAEKHAADFGADSQAAMKKALELFRNDMASKYKEFGFQG

SEQ ID NO: 7 - protein, 154 aa, Oryctolagus cuniculus
  source 1..154: note = Amino acid sequence of rabbit myoglobin
MGLSDAEWQLVLNVWGKVEADLAGHGQEVLIRLFHTHPETLEKFDKFKHLKSEDEMKASEDLKKHGNTVLTALGAILKKKGHHEAEIKPLAQSHATKHKIPVKYLEFISEAIIHVLHSKHPGDFGADAQAAMSKALELFRNDIAAQYKELGFQG

SEQ ID NO: 8 - protein, 154 aa, Bos taurus; identical to SEQ ID NO: 5
  source 1..154: note = Amino acid sequence of bovine myoglobin

SEQ ID NO: 9 - protein, 154 aa, Mus musculus
  source 1..154: note = Amino acid sequence of mouse myoglobin
MGLSDGEWQLVLNVWGKVEADLAGHGQEVLIGLFKTHPETLDKFDKFKNLKSEEDMKGSEDLKKHGCTVLTALGTILKKKGQHAAEIQPLAQSHATKHKIPVKYLEFISEIIIEVLKKRHSGDFGADAQGAMSKALELFRNDIAAKYKELGFQG

SEQ ID NO: 10 - protein, 154 aa, Rattus norvegicus
  source 1..154: note = Amino acid sequence of rat myoglobin
MGLSDGEWQMVLNIWGKVEGDLAGHGQEVLISLFKAHPETLEKFDKFKNLKSEEEMKSSEDLKKHGCTVLTALGTILKKKGQHAAEIQPLAQSHATKHKIPVKYLEFISEVIIQVLKKRYSGDFGADAQGAMSKALELFRNDIAAKYKELGFQG

SEQ ID NO: 11 - protein, 154 aa, Sus scrofa
  source 1..154: note = Amino acid sequence of tuna myoglobin
MGLSDGEWQLVLNVWGKVEADVAGHGQEVLIRLFKGHPETLEKFDKFKHLKSEDEMKASEDLKKHGNTVLTALGGILKKKGHHEAELTPLAQSHATKHKIPVKYLEFISEAIIQVLQSKHPGDFGADAQGAMSKALELFRNDMAAKYKELGFQG

SEQ ID NO: 12 - protein, 147 aa, Salmo salar
  source 1..147: note = Amino acid sequence of salmon myoglobin
MANYDMVLQCWEPVEADYNNHGGLVLSRLFAEHPETLTLFPKFAGIAAGDLSGNAAVAAHGATVLRKLGELLNARGDHAATLKSLATTHANKHKIPLKNFTLITNIICKVMGEKAGLDEAGQEALRQVMGVIIADINVTYMELGFAG

SEQ ID NO: 13 - protein, 146 aa, Sarda chiliensis
  source 1..146: note = Amino acid sequence of Blue bonito myoglobin
ADFDAVLKFWGPVEADYTSHGGLVLTRLFKEHPETQKLFPKFTGIAQADMAGNAAISAHGATVLKKLGELLKAKGNHAAILKPMANSHATKHKIPINNFKLISEIIVKVMQEKAGMDAGGQQALRNVMAAVIADLEANYKELGFSG

SEQ ID NO: 14 - protein, 147 aa, Xiphias gladius
  source 1..147: note = Amino acid sequence of sword fish myoglobin
MAEFEVVLKHWGPVEADYASHGNLVLTRLFTEHPDTQKLFPKFAGIAQGDMAGNAAISAHGATVLKKLGELLKAKGNHATTLKALATTHATKHKIPIKNFELIAEVIGKVMEEKAGLDSVGREALRDVMARVIADIDATYKELGFTG

SEQ ID NO: 15 - DNA, 6048 bp, synthetic construct
  source 1..6048: mol_type = other DNA; note = Nucleotide sequence of heterologous nucleic acid molecule comprising a nucleic acid sequence encoding a steppe mammoth myoglobin
aacatccaaagacgaaaggttgaatgaaacctttttgccatccgacatccacaggtccattctcacacataagtgccaaacgcaacaggaggggatacactagcagcagaccgttgcaaacgcaggacctccactcctcttctcctcaacacccacttttgccatcgaaaaaccagcccagttattgggcttgattggagctcgctcattccaattccttctattaggctactaacaccatgactttattagcctgtctatcctggcccccctggcgaggttcatgtttgtttatttccgaatgcaacaagctccgcattacacccgaacatcactccagatgagggctttctgagtgtggggtcaaatagtttcatgttccccaaatggcccaaaactgacagtttaaacgctgtcttggaacctaatatgacaaaagcgtgatctcatccaagatgaactaagtttggttcgttgaaatgctaacggccagttggtcaaaaagaaacttccaaaagtcgccataccgtttgtcttgtttggtattgattgacgaatgctcaaaaataatctcattaatgcttagcgcagtctctctatcgcttctgaaccccggtgcacctgtgccgaaacgcaaatggggaaacacccgctttttggatgattatgcattgtctccacattgtatgcttccaagattctggtgggaatactgctgatagcctaacgttcatgatcaaaatttaactgttctaacccctacttgacagcaatatataaacagaaggaagctgccctgtcttaaacctttttttttatcatcattattagcttactttcataattgcgactggttccaattgacaagcttttgattttaacgacttttaacgacaacttgagaagatcaaaaaacaactaattattcgaaacgatgagattcccatctattttcactgctgttttgttcgctgcttcttctgctttggctgctccagttaacactactactgaggatgaaactgctcaaattccagctgaagctgttattggttactctgatttggagggtgacttcgatgttgctgttttgccattctctaactctactaacaatggtttgttgttcattaacactactattgcttctattgctgctaaggaggaaggtgtttctttggagaagagagaagctgaggctggtttgtctgatggtgaatgggagttggttttgaagacttggggtaaagttgaggctgatattcctggtcatggtttggaggtttttgttagattgttcactggtcatccagaaactttggagaagttcgataagttcaaacatttgaagactgagggtgaaatgaaggcttctgaggatttgaaaaagcaaggtgttactgttttgactgctttgggtggtattttgaagaagaaaggtcaccatcaagctgaaattcaaccattggctcactctcatgctactaaacacaagattccaattaagtacttggagttcatttctgatgctattattcacgttttgcaatctaagcatccagctgaatttggtgctgatgctcaaggtgctatgaaaaaggctttggagttgttcagaaacgatattgctgctaaatacaaggagttgggtttccaaggttaagaattaattcgccttagacatgactgttcctcagttcaagttgggcacttacgagaagaccggtcttgctagattctaatcaagaggatgtcagaatgccatttgcctgagagatgcaggcttcatttttgatacttttttatttgtaacctatatagtataggattttttttgtcattttgtttcttctcgtacgagcttgctcctgatcagcctatctcgcagctgatgaatatcttgtggtaggggtttgggaaaatcattcgagtttgatgtttttcttggtatttcccactcctcttcagagtacagaagattaagtgagacgttcgtttgtgcaagcttatcgataagctttaatgcggtagtttatcacagttaaattgctaacgcagtcaggcaccgtgtatgaaatctaacaatgcgctcatcgtcatcctcggcaccgtcaccctggatgctgtaggcataggcttggttatgccggtactgccgggcctcttgcgggatatcgtccattccgacagcatcgccagtcactatggcgtgctgctagcgctatatgcgttgatgcaatttctatgcgcacccgttctcggagcactgtccgaccgctttggccgccgcccagtcctgctcgcttcgctacttggagccactatcgactacgcgatcatggcgaccacacccgtcctgtggatctatcgaatctaaatgtaagttaaaatctctaaataattaaataagtcccagtttctccatacgaaccttaacagcattgcggtgagcatctagaccttcaacagcagccagatccatcactgcttggccaatatgtttcagtccctcaggagttacgtcttgtgaagtgatgaacttctggaaggttgcagtgttaactccgctgtattgacgggcatatccgtacgttggcaaagtgtggttggtaccggaggagtaatctccacaactctctggagagtaggcaccaacaaacacagatccagcgtgttgtacttgatcaacataagaagaagcattctcgatttgcaggatcaagtgttcaggagcgtactgattggacatttccaaagcctgctcgtaggttgcaaccgatagggttgtagagtgtgcaatacacttgcgtacaatttcaacccttggcaactgcacagcttggttgtgaacagcatcttcaattctggcaagctccttgtctgtcatatcgacagccaacagaatcacctgggaatcaataccatgttcagcttgagacagaaggtctgaggcaacgaaatctggatcagcgtatttatcagcaataactagaacttcagaaggcccagcaggcatgtcaatactacacagggctgatgtgtcattttgaaccatcatcttggcagcagtaacgaactggtttcctggaccaaatattttgtcacacttaggaacagtttctgttccgtaagccatagcagctactgcctgggcgcctcctgctagcacgatacacttagcaccaaccttgtgggcaacgtagatgacttctggggtaagggtaccatccttcttaggtggagatgcaaaaacaatttctttgcaaccagcaactttggcaggaacacccagcatcagggaagtggaaggcagaattgcggttccaccaggaatatagaggccaactttctcaataggtcttgcaaaacgagagcagactacaccagggcaagtctcaacttgcaacgtctccgttagttgagcttcatggaatttcctgacgttatctatagagagatcaatggctctcttaacgttatctggcaattgcataagttcctctgggaaaggagcttctaacacaggtgtcttcaaagcgactccatcaaacttggcagttagttctaaaagggctttgtcaccattttgacgaacattgtcgacaattggtttgactaattccataatctgttccgttttctggataggacgacgaagggcatcttcaatttcttgtgaggaggccttagaaacgtcaattttgcacaattcaatacgaccttcagaagggacttctttaggtttggattcttctttaggttgttccttggtgtatcctggcttggcatctcctttccttctagtgacctttagggacttcatatccaggtttctctccacctcgtccaacgtcacaccgtacttggcacatctaactaatgcaaaataaaataagtcagcacattcccaggctatatcttccttggatttagcttctgcaagttcatcagcttcctccctaattttagcgttcaacaaaacttcgtcgtcaaataaccgtttggtataagaaccttctggagcattgctcttacgatcccacaaggtggcttccatggctctaagaccctttgattggccaaaacaggaagtgcgttccaagtgacagaaaccaacacctgtttgttcaaccacaaatttcaagcagtctccatcacaatccaattcgatacccagcaacttttgagttgctccagatgtagcacctttataccacaaaccgtgacgacgagattggtagactccagtttgtgtccttatagcctccggaatagactttttggacgagtacaccaggcccaacgagtaattagaagagtcagccaccaaagtagtgaatagaccatcggggcggtcagtagtcaaagacgccaacaaaatttcactgacagggaactttttgacatcttcagaaagttcgtattcagtagtcaattgccgagcatcaataatggggattataccagaagcaacagtggaagtcacatctaccaactttgcggtctcagaaaaagcataaacagttctactaccgccattagtgaaacttttcaaatcgcccagtggagaagaaaaaggcacagcgatactagcattagcgggcaaggatgcaactttatcaaccagggtcctatagataaccctagcgcctgggatcatcctttggacaactctttctgccaaatctaggtccaaaatcacttcattgataccattattgtacaacttgagcaagttgtcgatcagctcctcaaattggtcctctgtaacggatgactcaacttgcacattaacttgaagctcagtcgattgagtgaacttgatcaggttgtgcagctggtcagcagcatagggaaacacggcttttcctaccaaactcaaggaattatcaaactctgcaacacttgcgtatgcaggtagcaagggaaatgtcatacttgaagtcggacagtgagtgtagtcttgagaaattctgaagccgtatttttattatcagtgagtcagtcatcaggagatcctctacgccggacgcatcgtggccggcatcaccggcgccacaggtgcggttgctggcgcctatatcgccgacatcaccgatggggaagatcgggctcgccacttcgggctcatgagcgcttgtttcggcgtgggtatggtggcaggccccgtggccgggggactgttgggcgccatctccttgcatgcaccattccttgcggcggcggtgctcaacggcctcaacctactactgggctgcttcctaatgcaggagtcgcataagggagagcgtcgagtatctatgattggaagtatgggaatggtgatacccgcattcttcagtgtcttgaggtctcctatcagattatgcccaactaaagcaaccggaggaggagatttcatggtaaatttctctgacttttggtcatcagtagactcgaactgtgagactatctcggttatgacagcagaaatgtccttcttggagacagtaaatgaagtcccaccaataaagaaatccttgttatcaggaacaaacttcttgtttcgaactttttcggtgccttgaactataaaatgtagagtggatatgtcgggtaggaatggagcgggcaaatgcttaccttctggaccttcaagaggtatgtagggtttgtagatactgatgccaacttcagtgacaacgttgctatttcgttcaaaccattccgaatccagagaaatcaaagttgtttgtctactattgatccaagccagtgcggtcttgaaactgacaatagtgtgctcgtgttttgaggtcatctttgtatgaataaatctagtctttgatctaaataatcttgacgagccaaggcgataaatacccaaatctaaaactcttttaaaacgttaaaaggacaagtatgtctgcctgtattaaaccccaaatcagctcgtagtctgatcctcatcaacttgaggggcactatcttgttttagagaaatttgcggagatgcgatatcgagaaaaaggtacgctgattttaaacgtgaaatttatctcaagatct

SEQ ID NO: 16 - DNA, 6048 bp, synthetic construct
  source 1..6048: mol_type = other DNA; note = Nucleotide sequence of heterologous nucleic acid molecule comprising a nucleic acid sequence encoding a woolly mammoth myoglobin
aacatccaaagacgaaaggttgaatgaaacctttttgccatccgacatccacaggtccattctcacacataagtgccaaacgcaacaggaggggatacactagcagcagaccgttgcaaacgcaggacctccactcctcttctcctcaacacccacttttgccatcgaaaaaccagcccagttattgggcttgattggagctcgctcattccaattccttctattaggctactaacaccatgactttattagcctgtctatcctggcccccctggcgaggttcatgtttgtttatttccgaatgcaacaagctccgcattacacccgaacatcactccagatgagggctttctgagtgtggggtcaaatagtttcatgttccccaaatggcccaaaactgacagtttaaacgctgtcttggaacctaatatgacaaaagcgtgatctcatccaagatgaactaagtttggttcgttgaaatgctaacggccagttggtcaaaaagaaacttccaaaagtcgccataccgtttgtcttgtttggtattgattgacgaatgctcaaaaataatctcattaatgcttagcgcagtctctctatcgcttctgaaccccggtgcacctgtgccgaaacgcaaatggggaaacacccgctttttggatgattatgcattgtctccacattgtatgcttccaagattctggtgggaatactgctgatagcctaacgttcatgatcaaaatttaactgttctaacccctacttgacagcaatatataaacagaaggaagctgccctgtcttaaacctttttttttatcatcattattagcttactttcataattgcgactggttccaattgacaagcttttgattttaacgacttttaacgacaacttgagaagatcaaaaaacaactaattattcgaaacgatgagattcccatctattttcactgctgttttgttcgctgcttcttctgctttggctgctccagttaacactactactgaggatgaaactgctcaaattccagctgaagctgttattggttactctgatttggagggtgacttcgatgttgctgttttgccattctctaactctactaacaatggtttgttgttcattaacactactattgcttctattgctgctaaggaggaaggtgtttctttggagaagagagaagctgaggctggattgtccgacggtgaatgggagttggtccttaaaacttggggtaaggttgaagctgacatccctggccatggtttggaggtttttgttcgtctttttaccggacaccctgaaactttagagaaattcgataagtttaaacatctcaagaccgagggtgagatgaaagcatctgaagatttaaaaaagcagggtgtcacagtgctgacggctctaggagggattctgaagaagaaaggacatcaccaagcagaaattcagccacttgcccagagtcatgctactaagcacaagatccccattaagtacctagaattcatatcggatgcgatcatacatgtattgcaatcaaaacacccagctgaatttggcgcagatgcccaaggtgctatgaagaaagccttagaactgttcagaaacgacattgccgctaaatataaggagttgggattccaaggttaagaattaattcgccttagacatgactgttcctcagttcaagttgggcacttacgagaagaccggtcttgctagattctaatcaagaggatgtcagaatgccatttgcctgagagatgcaggcttcatttttgatacttttttatttgtaacctatatagtataggattttttttgtcattttgtttcttctcgtacgagcttgctcctgatcagcctatctcgcagctgatgaatatcttgtggtaggggtttgggaaaatcattcgagtttgatgtttttcttggtatttcccactcctcttcagagtacagaagattaagtgagacgttcgtttgtgcaagcttatcgataagctttaatgcggtagtttatcacagttaaattgctaacgcagtcaggcaccgtgtatgaaatctaacaatgcgctcatcgtcatcctcggcaccgtcaccctggatgctgtaggcataggcttggttatgccggtactgccgggcctcttgcgggatatcgtccattccgacagcatcgccagtcactatggcgtgctgctagcgctatatgcgttgatgcaatttctatgcgcacccgttctcggagcactgtccgaccgctttggccgccgcccagtcctgctcgcttcgctacttggagccactatcgactacgcgatcatggcgaccacacccgtcctgtggatctatcgaatctaaatgtaagttaaaatctctaaataattaaataagtcccagtttctccatacgaaccttaacagcattgcggtgagcatctagaccttcaacagcagccagatccatcactgcttggccaatatgtttcagtccctcaggagttacgtcttgtgaagtgatgaacttctggaaggttgcagtgttaactccgctgtattgacgggcatatccgtacgttggcaaagtgtggttggtaccggaggagtaatctccacaactctctggagagtaggcaccaacaaacacagatccagcgtgttgtacttgatcaacataagaagaagcattctcgatttgcaggatcaagtgttcaggagcgtactgattggacatttccaaagcctgctcgtaggttgcaaccgatagggttgtagagtgtgcaatacacttgcgtacaatttcaacccttggcaactgcacagcttggttgtgaacagcatcttcaattctggcaagctccttgtctgtcatatcgacagccaacagaatcacctgggaatcaataccatgttcagcttgagacagaaggtctgaggcaacgaaatctggatcagcgtatttatcagcaataactagaacttcagaaggcccagcaggcatgtcaatactacacagggctgatgtgtcattttgaaccatcatcttggcagcagtaacgaactggtttcctggaccaaatattttgtcacacttaggaacagtttctgttccgtaagccatagcagctactgcctgggcgcctcctgctagcacgatacacttagcaccaaccttgtgggcaacgtagatgacttctggggtaagggtaccatccttcttaggtggagatgcaaaaacaatttctttgcaaccagcaactttggcaggaacacccagcatcagggaagtggaaggcagaattgcggttccaccaggaatatagaggccaactttctcaataggtcttgcaaaacgagagcagactacaccagggcaagtctcaacttgcaacgtctccgttagttgagcttcatggaatttcctgacgttatctatagagagatcaatggctctcttaacgttatctggcaattgcataagttcctctgggaaaggagcttctaacacaggtgtcttcaaagcgactccatcaaacttggcagttagttctaaaagggctttgtcaccattttgacgaacattgtcgacaattggtttgactaattccataatctgttccgttttctggataggacgacgaagggcatcttcaatttcttgtgaggaggccttagaaacgtcaattttgcacaattcaatacgaccttcagaagggacttctttaggtttggattcttctttaggttgttccttggtgtatcctggcttggcatctcctttccttctagtgacctttagggacttcatatccaggtttctctccacctcgtccaacgtcacaccgtacttggcacatctaactaatgcaaaataaaataagtcagcacattcccaggctatatcttccttggatttagcttctgcaagttcatcagcttcctccctaattttagcgttcaacaaaacttcgtcgtcaaataaccgtttggtataagaaccttctggagcattgctcttacgatcccacaaggtggcttccatggctctaagaccctttgattggccaaaacaggaagtgcgttccaagtgacagaaaccaacacctgtttgttcaaccacaaatttcaagcagtctccatcacaatccaattcgatacccagcaacttttgagttgctccagatgtagcacctttataccacaaaccgtgacgacgagattggtagactccagtttgtgtccttatagcctccggaatagactttttggacgagtacaccaggcccaacgagtaattagaagagtcagccaccaaagtagtgaatagaccatcggggcggtcagtagtcaaagacgccaacaaaatttcactgacagggaactttttgacatcttcagaaagttcgtattcagtagtcaattgccgagcatcaataatggggattataccagaagcaacagtggaagtcacatctaccaactttgcggtctcagaaaaagcataaacagttctactaccgccattagtgaaacttttcaaatcgcccagtggagaagaaaaaggcacagcgatactagcattagcgggcaaggatgcaactttatcaaccagggtcctatagataaccctagcgcctgggatcatcctttggacaactctttctgccaaatctaggtccaaaatcacttcattgataccattattgtacaacttgagcaagttgtcgatcagctcctcaaattggtcctctgtaacggatgactcaacttgcacattaacttgaagctcagtcgattgagtgaacttgatcaggttgtgcagctggtcagcagcatagggaaacacggcttttcctaccaaactcaaggaattatcaaactctgcaacacttgcgtatgcaggtagcaagggaaatgtcatacttgaagtcggacagtgagtgtagtcttgagaaattctgaagccgtatttttattatcagtgagtcagtcatcaggagatcctctacgccggacgcatcgtggccggcatcaccggcgccacaggtgcggttgctggcgcctatatcgccgacatcaccgatggggaagatcgggctcgccacttcgggctcatgagcgcttgtttcggcgtgggtatggtggcaggccccgtggccgggggactgttgggcgccatctccttgcatgcaccattccttgcggcggcggtgctcaacggcctcaacctactactgggctgcttcctaatgcaggagtcgcataagggagagcgtcgagtatctatgattggaagtatgggaatggtgatacccgcattcttcagtgtcttgaggtctcctatcagattatgcccaactaaagcaaccggaggaggagatttcatggtaaatttctctgacttttggtcatcagtagactcgaactgtgagactatctcggttatgacagcagaaatgtccttcttggagacagtaaatgaagtcccaccaataaagaaatccttgttatcaggaacaaacttcttgtttcgaactttttcggtgccttgaactataaaatgtagagtggatatgtcgggtaggaatggagcgggcaaatgcttaccttctggaccttcaagaggtatgtagggtttgtagatactgatgccaacttcagtgacaacgttgctatttcgttcaaaccattccgaatccagagaaatcaaagttgtttgtctactattgatccaagccagtgcggtcttgaaactgacaatagtgtgctcgtgttttgaggtcatctttgtatgaataaatctagtctttgatctaaataatcttgacgagccaaggcgataaatacccaaatctaaaactcttttaaaacgttaaaaggacaagtatgtctgcctgtattaaaccccaaatcagctcgtagtctgatcctcatcaacttgaggggcactatcttgttttagagaaatttgcggagatgcgatatcgagaaaaaggtacgctgattttaaacgtgaaatttatctcaagatct

SEQ ID NO: 17 - DNA, 6048 bp, synthetic construct
  source 1..6048: mol_type = other DNA; note = Nucleotide sequence of heterologous nucleic acid molecule comprising a nucleic acid sequence encoding a pig myoglobin
aacatccaaagacgaaaggttgaatgaaacctttttgccatccgacatccacaggtccattctcacacataagtgccaaacgcaacaggaggggatacactagcagcagaccgttgcaaacgcaggacctccactcctcttctcctcaacacccacttttgccatcgaaaaaccagcccagttattgggcttgattggagctcgctcattccaattccttctattaggctactaacaccatgactttattagcctgtctatcctggcccccctggcgaggttcatgtttgtttatttccgaatgcaacaagctccgcattacacccgaacatcactccagatgagggctttctgagtgtggggtcaaatagtttcatgttccccaaatggcccaaaactgacagtttaaacgctgtcttggaacctaatatgacaaaagcgtgatctcatccaagatgaactaagtttggttcgttgaaatgctaacggccagttggtcaaaaagaaacttccaaaagtcgccataccgtttgtcttgtttggtattgattgacgaatgctcaaaaataatctcattaatgcttagcgcagtctctctatcgcttctgaaccccggtgcacctgtgccgaaacgcaaatggggaaacacccgctttttggatgattatgcattgtctccacattgtatgcttccaagattctggtgggaatactgctgatagcctaacgttcatgatcaaaatttaactgttctaacccctacttgacagcaatatataaacagaaggaagctgccctgtcttaaacctttttttttatcatcattattagcttactttcataattgcgactggttccaattgacaagcttttgattttaacgacttttaacgacaacttgagaagatcaaaaaacaactaattattcgaaacgatgagattcccatctattttcactgctgttttgttcgctgcttcttctgctttggctgctccagttaacactactactgaggatgaaactgctcaaattccagctgaagctgttattggttactctgatttggagggtgacttcgatgttgctgttttgccattctctaattctactaacaatggtttgttgttcattaacactactattgcttctattgctgctaaggaagagggtgtttctttggagaagagagaagctgaggctggtttgtctgatggtgaatggcaattggttttgaacgtttggggtaaagttgaggctgatgttgctggtcatggtcaagaggttttgattagattgttcaagggtcatccagaaactttggagaaatttgataagttcaagcacttgaagtctgaagatgagatgaaggcttctgaggatttgaagaaacacggtaacactgttttgactgctttgggtggtattttgaaaaagaaaggtcaccatgaagctgagttgactccattggctcaatctcatgctactaagcacaagattccagttaaatacttggagtttatttctgaggctattattcaagttttgcaatctaagcatcctggtgacttcggtgctgatgctcaaggtgctatgtctaaggctttggagttgttcagaaacgatatggctgctaagtacaaggagttgggtttccaaggttaagaattaattcgccttagacatgactgttcctcagttcaagttgggcacttacgagaagaccggtcttgctagattctaatcaagaggatgtcagaatgccatttgcctgagagatgcaggcttcatttttgatacttttttatttgtaacctatatagtataggattttttttgtcattttgtttcttctcgtacgagcttgctcctgatcagcctatctcgcagctgatgaatatcttgtggtaggggtttgggaaaatcattcgagtttgatgtttttcttggtatttcccactcctcttcagagtacagaagattaagtgagacgttcgtttgtgcaagcttatcgataagctttaatgcggtagtttatcacagttaaattgctaacgcagtcaggcaccgtgtatgaaatctaacaatgcgctcatcgtcatcctcggcaccgtcaccctggatgctgtaggcataggcttggttatgccggtactgccgggcctcttgcgggatatcgtccattccgacagcatcgccagtcactatggcgtgctgctagcgctatatgcgttgatgcaatttctatgcgcacccgttctcggagcactgtccgaccgctttggccgccgcccagtcctgctcgcttcgctacttggagccactatcgactacgcgatcatggcgaccacacccgtcctgtggatctatcgaatctaaatgtaagttaaaatctctaaataattaaataagtcccagtttctccatacgaaccttaacagcattgcggtgagcatctagaccttcaacagcagccagatccatcactgcttggccaatatgtttcagtccctcaggagttacgtcttgtgaagtgatgaacttctggaaggttgcagtgttaactccgctgtattgacgggcatatccgtacgttggcaaagtgtggttggtaccggaggagtaatctccacaactctctggagagtaggcaccaacaaacacagatccagcgtgttgtacttgatcaacataagaagaagcattctcgatttgcaggatcaagtgttcaggagcgtactgattggacatttccaaagcctgctcgtaggttgcaaccgatagggttgtagagtgtgcaatacacttgcgtacaatttcaacccttggcaactgcacagcttggttgtgaacagcatcttcaattctggcaagctccttgtctgtcatatcgacagccaacagaatcacctgggaatcaataccatgttcagcttgagacagaaggtctgaggcaacgaaatctggatcagcgtatttatcagcaataactagaacttcagaaggcccagcaggcatgtcaatactacacagggctgatgtgtcattttgaaccatcatcttggcagcagtaacgaactggtttcctggaccaaatattttgtcacacttaggaacagtttctgttccgtaagccatagcagctactgcctgggcgcctcctgctagcacgatacacttagcaccaaccttgtgggcaacgtagatgacttctggggtaagggtaccatccttcttaggtggagatgcaaaaacaatttctttgcaaccagcaactttggcaggaacacccagcatcagggaagtggaaggcagaattgcggttccaccaggaatatagaggccaactttctcaataggtcttgcaaaacgagagcagactacaccagggcaagtctcaacttgcaacgtctccgttagttgagcttcatggaatttcctgacgttatctatagagagatcaatggctctcttaacgttatctggcaattgcataagttcctctgggaaaggagcttctaacacaggtgtcttcaaagcgactccatcaaacttggcagttagttctaaaagggctttgtcaccattttgacgaacattgtcgacaattggtttgactaattccataatctgttccgttttctggataggacgacgaagggcatcttcaatttcttgtgaggaggccttagaaacgtcaattttgcacaattcaatacgaccttcagaagggacttctttaggtttggattcttctttaggttgttccttggtgtatcctggcttggcatctcctttccttctagtgacctttagggacttcatatccaggtttctctccacctcgtccaacgtcacaccgtacttggcacatctaactaatgcaaaataaaataagtcagcacattcccaggctatatcttccttggatttagcttctgcaagttcatcagcttcctccctaattttagcgttcaacaaaacttcgtcgtcaaataaccgtttggtataagaaccttctggagcattgctcttacgatcccacaaggtggcttccatggctctaagaccctttgattggccaaaacaggaagtgcgttccaagtgacagaaaccaacacctgtttgttcaaccacaaatttcaagcagtctccatcacaatccaattcgatacccagcaacttttgagttgctccagatgtagcacctttataccacaaaccgtgacgacgagattggtagactccagtttgtgtccttatagcctccggaatagactttttggacgagtacaccaggcccaacgagtaattagaagagtcagccaccaaagtagtgaatagaccatcggggcggtcagtagtcaaagacgccaacaaaatttcactgacagggaactttttgacatcttcagaaagttcgtattcagtagtcaattgccgagcatcaataatggggattataccagaagcaacagtggaagtcacatctaccaactttgcggtctcagaaaaagcataaacagttctactaccgccattagtgaaacttttcaaatcgcccagtggagaagaaaaaggcacagcgatactagcattagcgggcaaggatgcaactttatcaaccagggtcctatagataaccctagcgcctgggatcatcctttggacaactctttctgccaaatctaggtccaaaatcacttcattgataccattattgtacaacttgagcaagttgtcgatcagctcctcaaattggtcctctgtaacggatgactcaacttgcacattaacttgaagctcagtcgattgagtgaacttgatcaggttgtgcagctggtcagcagcatagggaaacacggcttttcctaccaaactcaaggaattatcaaactctgcaacacttgcgtatgcaggtagcaagggaaatgtcatacttgaagtcggacagtgagtgtagtcttgagaaattctgaagccgtatttttattatcagtgagtcagtcatcaggagatcctctacgccggacgcatcgtggccggcatcaccggcgccacaggtgcggttgctggcgcctatatcgccgacatcaccgatggggaagatcgggctcgccacttcgggctcatgagcgcttgtttcggcgtgggtatggtggcaggccccgtggccgggggactgttgggcgccatctccttgcatgcaccattccttgcggcggcggtgctcaacggcctcaacctactactgggctgcttcctaatgcaggagtcgcataagggagagcgtcgagtatctatgattggaagtatgggaatggtgatacccgcattcttcagtgtcttgaggtctcctatcagattatgcccaactaaagcaaccggaggaggagatttcatggtaaatttctctgacttttggtcatcagtagactcgaactgtgagactatctcggttatgacagcagaaatgtccttcttggagacagtaaatgaagtcccaccaataaagaaatccttgttatcaggaacaaacttcttgtttcgaactttttcggtgccttgaactataaaatgtagagtggatatgtcgggtaggaatggagcgggcaaatgcttaccttctggaccttcaagaggtatgtagggtttgtagatactgatgccaacttcagtgacaacgttgctatttcgttcaaaccattccgaatccagagaaatcaaagttgtttgtctactattgatccaagccagtgcggtcttgaaactgacaatagtgtgctcgtgttttgaggtcatctttgtatgaataaatctagtctttgatctaaataatcttgacgagccaaggcgataaatacccaaatctaaaactcttttaaaacgttaaaaggacaagtatgtctgcctgtattaaaccccaaatcagctcgtagtctgatcctcatcaacttgaggggcactatcttgttttagagaaatttgcggagatgcgatatcgagaaaaaggtacgctgattttaaacgtgaaatttatctcaagatct

SEQ ID NO: 18 - DNA, 6048 bp, synthetic construct
  source 1..6048: mol_type = other DNA; note = Nucleotide sequence of heterologous nucleic acid molecule comprising a nucleic acid sequence encoding a sheep myoglobin
aacatccaaagacgaaaggttgaatgaaacctttttgccatccgacatccacaggtccattctcacacataagtgccaaacgcaacaggaggggatacactagcagcagaccgttgcaaacgcaggacctccactcctcttctcctcaacacccacttttgccatcgaaaaaccagcccagttattgggcttgattggagctcgctcattccaattccttctattaggctactaacaccatgactttattagcctgtctatcctggcccccctggcgaggttcatgtttgtttatttccgaatgcaacaagctccgcattacacccgaacatcactccagatgagggctttctgagtgtggggtcaaatagtttcatgttccccaaatggcccaaaactgacagtttaaacgctgtcttggaacctaatatgacaaaagcgtgatctcatccaagatgaactaagtttggttcgttgaaatgctaacggccagttggtcaaaaagaaacttccaaaagtcgccataccgtttgtcttgtttggtattgattgacgaatgctcaaaaataatctcattaatgcttagcgcagtctctctatcgcttctgaaccccggtgcacctgtgccgaaacgcaaatggggaaacacccgctttttggatgattatgcattgtctccacattgtatgcttccaagattctggtgggaatactgctgatagcctaacgttcatgatcaaaatttaactgttctaacccctacttgacagcaatatataaacagaaggaagctgccctgtcttaaacctttttttttatcatcattattagcttactttcataattgcgactggttccaattgacaagcttttgattttaacgacttttaacgacaacttgagaagatcaaaaaacaactaattattcgaaacgatgagattcccatctattttcactgctgttttgttcgctgcttcttctgctttggctgctcctgttaatactactactgaggatgaaactgctcaaattcctgctgaagctgttattggttattctgatttggagggtgacttcgatgttgctgttttgcctttctctaactctactaataacggtttgttgttcattaacactactattgcttctattgctgctaaggaagagggtgtttctttggaaaagagagaggctgaagctggtttgtctgatggtgaatggcaattggttttgaacgcttggggtaaagttgaggctgatgttgctggtcatggtcaagaagttttgattagattgttcactggtcaccctgaaactttggagaagtttgataagttcaaacacttgaagactgaggctgaaatgaaggcttctgaggatttgaaaaagcatggtaacactgttttgactgctttgggtggtattttgaagaagaaaggtcaccatgaagctgaggttaagcacttggctgaatctcacgctaacaagcacaaaattcctgttaagtacttggagttcatttctgatgctattattcatgttttgcacgctaagcatccatctgatttcggtgctgatgctcaaggtgctatgtctaaggctttggaattgttcagaaacgatatggctgctcaatacaaggttttgggtttccaaggttaagaattaattcgccttagacatgactgttcctcagttcaagttgggcacttacgagaagaccggtcttgctagattctaatcaagaggatgtcagaatgccatttgcctgagagatgcaggcttcatttttgatacttttttatttgtaacctatatagtataggattttttttgtcattttgtttcttctcgtacgagcttgctcctgatcagcctatctcgcagctgatgaatatcttgtggtaggggtttgggaaaatcattcgagtttgatgtttttcttggtatttcccactcctcttcagagtacagaagattaagtgagacgttcgtttgtgcaagcttatcgataagctttaatgcggtagtttatcacagttaaattgctaacgcagtcaggcaccgtgtatgaaatctaacaatgcgctcatcgtcatcctcggcaccgtcaccctggatgctgtaggcataggcttggttatgccggtactgccgggcctcttgcgggatatcgtccattccgacagcatcgccagtcactatggcgtgctgctagcgctatatgcgttgatgcaatttctatgcgcacccgttctcggagcactgtccgaccgctttggccgccgcccagtcctgctcgcttcgctacttggagccactatcgactacgcgatcatggcgaccacacccgtcctgtggatctatcgaatctaaatgtaagttaaaatctctaaataattaaataagtcccagtttctccatacgaaccttaacagcattgcggtgagcatctagaccttcaacagcagccagatccatcactgcttggccaatatgtttcagtccctcaggagttacgtcttgtgaagtgatgaacttctggaaggttgcagtgttaactccgctgtattgacgggcatatccgtacgttggcaaagtgtggttggtaccggaggagtaatctccacaactctctggagagtaggcaccaacaaacacagatccagcgtgttgtacttgatcaacataagaagaagcattctcgatttgcaggatcaagtgttcaggagcgtactgattggacatttccaaagcctgctcgtaggttgcaaccgatagggttgtagagtgtgcaatacacttgcgtacaatttcaacccttggcaactgcacagcttggttgtgaacagcatcttcaattctggcaagctccttgtctgtcatatcgacagccaacagaatcacctgggaatcaataccatgttcagcttgagacagaaggtctgaggcaacgaaatctggatcagcgtatttatcagcaataactagaacttcagaaggcccagcaggcatgtcaatactacacagggctgatgtgtcattttgaaccatcatcttggcagcagtaacgaactggtttcctggaccaaatattttgtcacacttaggaacagtttctgttccgtaagccatagcagctactgcctgggcgcctcctgctagcacgatacacttagcaccaaccttgtgggcaacgtagatgacttctggggtaagggtaccatccttcttaggtggagatgcaaaaacaatttctttgcaaccagcaactttggcaggaacacccagcatcagggaagtggaaggcagaattgcggttccaccaggaatatagaggccaactttctcaataggtcttgcaaaacgagagcagactacaccagggcaagtctcaacttgcaacgtctccgttagttgagcttcatggaatttcctgacgttatctatagagagatcaatggctctcttaacgttatctggcaattgcataagttcctctgggaaaggagcttctaacacaggtgtcttcaaagcgactccatcaaacttggcagttagttctaaaagggctttgtcaccattttgacgaacattgtcgacaattggtttgactaattccataatctgttccgttttctggataggacgacgaagggcatcttcaatttcttgtgaggaggccttagaaacgtcaattttgcacaattcaatacgaccttcagaagggacttctttaggtttggattcttctttaggttgttccttggtgtatcctggcttggcatctcctttccttctagtgacctttagggacttcatatccaggtttctctccacctcgtccaacgtcacaccgtacttggcacatctaactaatgcaaaataaaataagtcagcacattcccaggctatatcttccttggatttagcttctgcaagttcatcagcttcctccctaattttagcgttcaacaaaacttcgtcgtcaaataaccgtttggtataagaaccttctggagcattgctcttacgatcccacaaggtggcttccatggctctaagaccctttgattggccaaaacaggaagtgcgttccaagtgacagaaaccaacacctgtttgttcaaccacaaatttcaagcagtctccatcacaatccaattcgatacccagcaacttttgagttgctccagatgtagcacctttataccacaaaccgtgacgacgagattggtagactccagtttgtgtccttatagcctccggaatagactttttggacgagtacaccaggcccaacgagtaattagaagagtcagccaccaaagtagtgaatagaccatcggggcggtcagtagtcaaagacgccaacaaaatttcactgacagggaactttttgacatcttcagaaagttcgtattcagtagtcaattgccgagcatcaataatggggattataccagaagcaacagtggaagtcacatctaccaactttgcggtctcagaaaaagcataaacagttctactaccgccattagtgaaacttttcaaatcgcccagtggagaagaaaaaggcacagcgatactagcattagcgggcaaggatgcaactttatcaaccagggtcctatagataaccctagcgcctgggatcatcctttggacaactctttctgccaaatctaggtccaaaatcacttcattgataccattattgtacaacttgagcaagttgtcgatcagctcctcaaattggtcctctgtaacggatgactcaacttgcacattaacttgaagctcagtcgattgagtgaacttgatcaggttgtgcagctggtcagcagcatagggaaacacggcttttcctaccaaactcaaggaattatcaaactctgcaacacttgcgtatgcaggtagcaagggaaatgtcatacttgaagtcggacagtgagtgtagtcttgagaaattctgaagccgtatttttattatcagtgagtcagtcatcaggagatcctctacgccggacgcatcgtggccggcatcaccggcgccacaggtgcggttgctggcgcctatatcgccgacatcaccgatggggaagatcgggctcgccacttcgggctcatgagcgcttgtttcggcgtgggtatggtggcaggccccgtggccgggggactgttgggcgccatctccttgcatgcaccattccttgcggcggcggtgctcaacggcctcaacctactactgggctgcttcctaatgcaggagtcgcataagggagagcgtcgagtatctatgattggaagtatgggaatggtgatacccgcattcttcagtgtcttgaggtctcctatcagattatgcccaactaaagcaaccggaggaggagatttcatggtaaatttctctgacttttggtcatcagtagactcgaactgtgagactatctcggttatgacagcagaaatgtccttcttggagacagtaaatgaagtcccaccaataaagaaatccttgttatcaggaacaaacttcttgtttcgaactttttcggtgccttgaactataaaatgtagagtggatatgtcgggtaggaatggagcgggcaaatgcttaccttctggaccttcaagaggtatgtagggtttgtagatactgatgccaacttcagtgacaacgttgctatttcgttcaaaccattccgaatccagagaaatcaaagttgtttgtctactattgatccaagccagtgcggtcttgaaactgacaatagtgtgctcgtgttttgaggtcatctttgtatgaataaatctagtctttgatctaaataatcttgacgagccaaggcgataaatacccaaatctaaaactcttttaaaacgttaaaaggacaagtatgtctgcctgtattaaaccccaaatcagctcgtagtctgatcctcatcaacttgaggggcactatcttgttttagagaaatttgcggagatgcgatatcgagaaaaaggtacgctgattttaaacgtgaaatttatctcaagatct

SEQ ID NO: 19 - DNA, 6048 bp, synthetic construct
  source 1..6048: mol_type = other DNA; note = Nucleotide sequence of heterologous nucleic acid molecule comprising a nucleic acid sequence encoding a cow myoglobin
aacatccaaagacgaaaggttgaatgaaacctttttgccatccgacatccacaggtccattctcacacataagtgccaaacgcaacaggaggggatacactagcagcagaccgttgcaaacgcaggacctccactcctcttctcctcaacacccacttttgccatcgaaaaaccagcccagttattgggcttgattggagctcgctcattccaattccttctattaggctactaacaccatgactttattagcctgtctatcctggcccccctggcgaggttcatgtttgtttatttccgaatgcaacaagctccgcattacacccgaacatcactccagatgagggctttctgagtgtggggtcaaatagtttcatgttccccaaatggcccaaaactgacagtttaaacgctgtcttggaacctaatatgacaaaagcgtgatctcatccaagatgaactaagtttggttcgttgaaatgctaacggccagttggtcaaaaagaaacttccaaaagtcgccataccgtttgtcttgtttggtattgattgacgaatgctcaaaaataatctcattaatgcttagcgcagtctctctatcgcttctgaaccccggtgcacctgtgccgaaacgcaaatggggaaacacccgctttttggatgattatgcattgtctccacattgtatgcttccaagattctggtgggaatactgctgatagcctaacgttcatgatcaaaatttaactgttctaacccctacttgacagcaatatataaacagaaggaagctgccctgtcttaaacctttttttttatcatcattattagcttactttcataattgcgactggttccaattgacaagcttttgattttaacgacttttaacgacaacttgagaagatcaaaaaacaactaattattcgaaacgatgagattcccatctattttcactgctgttttgttcgctgcttcttctgctttggctgctccagttaacactactactgaggatgaaactgctcaaattccagctgaagctgttattggttactctgatttggagggtgacttcgatgttgctgttttgccattctctaactctactaacaatggtttgttgttcattaacactactattgcttctattgctgctaaggaggaaggtgtttctttggagaagagagaagctgaggctggtttgtctgatggtgaatggcaattggttttgaacgcttggggtaaagttgaggctgatgttgctggtcatggtcaagaggttttgattagattgttcactggtcatccagaaactttggagaagtttgataaattcaagcacttgaagactgaagctgagatgaaggcttctgaggatttgaaaaagcacggtaacactgttttgactgctttgggtggtattttgaagaaaaagggtcaccatgaggctgaagttaagcacttggctgaatctcatgctaacaagcacaaaattcctgttaagtacttggagttcatttctgatgctattattcacgttttgcatgctaagcacccatctgatttcggtgctgatgctcaagctgctatgtctaaggctttggagttgtttagaaacgatatggctgctcaatacaaggttttgggtttccacggttaagaattaattcgccttagacatgactgttcctcagttcaagttgggcacttacgagaagaccggtcttgctagattctaatcaagaggatgtcagaatgccatttgcctgagagatgcaggcttcatttttgatacttttttatttgtaacctatatagtataggattttttttgtcattttgtttcttctcgtacgagcttgctcctgatcagcctatctcgcagctgatgaatatcttgtggtaggggtttgggaaaatcattcgagtttgatgtttttcttggtatttcccactcctcttcagagtacagaagattaagtgagacgttcgtttgtgcaagcttatcgataagctttaatgcggtagtttatcacagttaaattgctaacgcagtcaggcaccgtgtatgaaatctaacaatgcgctcatcgtcatcctcggcaccgtcaccctggatgctgtaggcataggcttggttatgccggtactgccgggcctcttgcgggatatcgtccattccgacagcatcgccagtcactatggcgtgctgctagcgctatatgcgttgatgcaatttctatgcgcacccgttctcggagcactgtccgaccgctttggccgccgcccagtcctgctcgcttcgctacttggagccactatcgactacgcgatcatggcgaccacacccgtcctgtggatctatcgaatctaaatgtaagttaaaatctctaaataattaaataagtcccagtttctccatacgaaccttaacagcattgcggtgagcatctagaccttcaacagcagccagatccatcactgcttggccaatatgtttcagtccctcaggagttacgtcttgtgaagtgatgaacttctggaaggttgcagtgttaactccgctgtattgacgggcatatccgtacgttggcaaagtgtggttggtaccggaggagtaatctccacaactctctggagagtaggcaccaacaaacacagatccagcgtgttgtacttgatcaacataagaagaagcattctcgatttgcaggatcaagtgttcaggagcgtactgattggacatttccaaagcctgctcgtaggttgcaaccgatagggttgtagagtgtgcaatacacttgcgtacaatttcaacccttggcaactgcacagcttggttgtgaacagcatcttcaattctggcaagctccttgtctgtcatatcgacagccaacagaatcacctgggaatcaataccatgttcagcttgagacagaaggtctgaggcaacgaaatctggatcagcgtatttatcagcaataactagaacttcagaaggcccagcaggcatgtcaatactacacagggctgatgtgtcattttgaaccatcatcttggcagcagtaacgaactggtttcctggaccaaatattttgtcacacttaggaacagtttctgttccgtaagccatagcagctactgcctgggcgcctcctgctagcacgatacacttagcaccaaccttgtgggcaacgtagatgacttctggggtaagggtaccatccttcttaggtggagatgcaaaaacaatttctttgcaaccagcaactttggcaggaacacccagcatcagggaagtggaaggcagaattgcggttccaccaggaatatagaggccaactttctcaataggtcttgcaaaacgagagcagactacaccagggcaagtctcaacttgcaacgtctccgttagttgagcttcatggaatttcctgacgttatctatagagagatcaatggctctcttaacgttatctggcaattgcataagttcctctgggaaaggagcttctaacacaggtgtcttcaaagcgactccatcaaacttggcagttagttctaaaagggctttgtcaccattttgacgaacattgtcgacaattggtttgactaattccataatctgttccgttttctggataggacgacgaagggcatcttcaatttcttgtgaggaggccttagaaacgtcaattttgcacaattcaatacgaccttcagaagggacttctttaggtttggattcttctttaggttgttccttggtgtatcctggcttggcatctcctttccttctagtgacctttagggacttcatatccaggtttctctccacctcgtccaacgtcacaccgtacttggcacatctaactaatgcaaaataaaataagtcagcacattcccaggctatatcttccttggatttagcttctgcaagttcatcagcttcctccctaattttagcgttcaacaaaacttcgtcgtcaaataaccgtttggtataagaaccttctggagcattgctcttacgatcccacaaggtggcttccatggctctaagaccctttgattggccaaaacaggaagtgcgttccaagtgacagaaaccaacacctgtttgttcaaccacaaatttcaagcagtctccatcacaatccaattcgatacccagcaacttttgagttgctccagatgtagcacctttataccacaaaccgtgacgacgagattggtagactccagtttgtgtccttatagcctccggaatagactttttggacgagtacaccaggcccaacgagtaattagaagagtcagccaccaaagtagtgaatagaccatcggggcggtcagtagtcaaagacgccaacaaaatttcactgacagggaactttttgacatcttcagaaagttcgtattcagtagtcaattgccgagcatcaataatggggattataccagaagcaacagtggaagtcacatctaccaactttgcggtctcagaaaaagcataaacagttctactaccgccattagtgaaacttttcaaatcgcccagtggagaagaaaaaggcacagcgatactagcattagcgggcaaggatgcaactttatcaaccagggtcctatagataaccctagcgcctgggatcatcctttggacaactctttctgccaaatctaggtccaaaatcacttcattgataccattattgtacaacttgagcaagttgtcgatcagctcctcaaattggtcctctgtaacggatgactcaacttgcacattaacttgaagctcagtcgattgagtgaacttgatcaggttgtgcagctggtcagcagcatagggaaacacggcttttcctaccaaactcaaggaattatcaaactctgcaacacttgcgtatgcaggtagcaagggaaatgtcatacttgaagtcggacagtgagtgtagtcttgagaaattctgaagccgtatttttattatcagtgagtcagtcatcaggagatcctctacgccggacgcatcgtggccggcatcaccggcgccacaggtgcggttgctggcgcctatatcgccgacatcaccgatggggaagatcgggctcgccacttcgggctcatgagcgcttgtttcggcgtgggtatggtggcaggccccgtggccgggggactgttgggcgccatctccttgcatgcaccattccttgcggcggcggtgctcaacggcctcaacctactactgggctgcttcctaatgcaggagtcgcataagggagagcgtcgagtatctatgattggaagtatgggaatggtgatacccgcattcttcagtgtcttgaggtctcctatcagattatgcccaactaaagcaaccggaggaggagatttcatggtaaatttctctgacttttggtcatcagtagactcgaactgtgagactatctcggttatgacagcagaaatgtccttcttggagacagtaaatgaagtcccaccaataaagaaatccttgttatcaggaacaaacttcttgtttcgaactttttcggtgccttgaactataaaatgtagagtggatatgtcgggtaggaatggagcgggcaaatgcttaccttctggaccttcaagaggtatgtagggtttgtagatactgatgccaacttcagtgacaacgttgctatttcgttcaaaccattccgaatccagagaaatcaaagttgtttgtctactattgatccaagccagtgcggtcttgaaactgacaatagtgtgctcgtgttttgaggtcatctttgtatgaataaatctagtctttgatctaaataatcttgacgagccaaggcgataaatacccaaatctaaaactcttttaaaacgttaaaaggacaagtatgtctgcctgtattaaaccccaaatcagctcgtagtctgatcctcatcaacttgaggggcactatcttgttttagagaaatttgcggagatgcgatatcgagaaaaaggtacgctgattttaaacgtgaaatttatctcaagatct

SEQ ID NO: 20 - DNA, 6048 bp, synthetic construct
  source 1..6048: mol_type = other DNA; note = Nucleotide sequence of heterologous nucleic acid molecule comprising a nucleic acid sequence encoding a chicken myoglobin
aacatccaaagacgaaaggttgaatgaaacctttttgccatccgacatccacaggtccattctcacacataagtgccaaacgcaacaggaggggatacactagcagcagaccgttgcaaacgcaggacctccactcctcttctcctcaacacccacttttgccatcgaaaaaccagcccagttattgggcttgattggagctcgctcattccaattccttctattaggctactaacaccatgactttattagcctgtctatcctggcccccctggcgaggttcatgtttgtttatttccgaatgcaacaagctccgcattacacccgaacatcactccagatgagggctttctgagtgtggggtcaaatagtttcatgttccccaaatggcccaaaactgacagtttaaacgctgtcttggaacctaatatgacaaaagcgtgatctcatccaagatgaactaagtttggttcgttgaaatgctaacggccagttggtcaaaaagaaacttccaaaagtcgccataccgtttgtcttgtttggtattgattgacgaatgctcaaaaataatctcattaatgcttagcgcagtctctctatcgcttctgaaccccggtgcacctgtgccgaaacgcaaatggggaaacacccgctttttggatgattatgcattgtctccacattgtatgcttccaagattctggtgggaatactgctgatagcctaacgttcatgatcaaaatttaactgttctaacccctacttgacagcaatatataaacagaaggaagctgccctgtcttaaacctttttttttatcatcattattagcttactttcataattgcgactggttccaattgacaagcttttgattttaacgacttttaacgacaacttgagaagatcaaaaaacaactaattattcgaaacgatgagattcccatctattttcactgctgttttgttcgctgcttcttctgctttggctgctccagttaacactactactgaagatgagactgctcaaattcctgctgaagctgttattggttactctgatttggagggtgacttcgatgttgctgttttgcctttttctaactctactaacaatggtttgttgttcattaacactactattgcttctattgctgctaaggaagagggtgtttctttggagaaaagagaggctgaagctggtttgtctgatcaagaatggcaacaagttttgactatttggggtaaagttgaggctgatattgctggtcatggtcacgaggttttgatgagattgttccatgatcacccagaaactttggatagattcgataagttcaagggtttgaaaactccagatcaaatgaagggttctgaggatttgaagaaacacggtgctactgttttgactcaattgggtaaaattttgaagcaaaaaggtaaccatgagtctgaattgaagccattggctcaaactcacgctactaagcacaagattcctgttaagtacttggagttcatttctgaggttattattaaggttattgctgaaaagcatgctgctgatttcggtgctgattctcaagctgctatgaaaaaggctttggaattgttcagaaacgatatggcttctaaatacaaggagttcggttttcaaggttaagaattaattcgccttagacatgactgttcctcagttcaagttgggcacttacgagaagaccggtcttgctagattctaatcaagaggatgtcagaatgccatttgcctgagagatgcaggcttcatttttgatacttttttatttgtaacctatatagtataggattttttttgtcattttgtttcttctcgtacgagcttgctcctgatcagcctatctcgcagctgatgaatatcttgtggtaggggtttgggaaaatcattcgagtttgatgtttttcttggtatttcccactcctcttcagagtacagaagattaagtgagacgttcgtttgtgcaagcttatcgataagctttaatgcggtagtttatcacagttaaattgctaacgcagtcaggcaccgtgtatgaaatctaacaatgcgctcatcgtcatcctcggcaccgtcaccctggatgctgtaggcataggcttggttatgccggtactgccgggcctcttgcgggatatcgtccattccgacagcatcgccagtcactatggcgtgctgctagcgctatatgcgttgatgcaatttctatgcgcacccgttctcggagcactgtccgaccgctttggccgccgcccagtcctgctcgcttcgctacttggagccactatcgactacgcgatcatggcgaccacacccgtcctgtggatctatcgaatctaaatgtaagttaaaatctctaaataattaaataagtcccagtttctccatacgaaccttaacagcattgcggtgagcatctagaccttcaacagcagccagatccatcactgcttggccaatatgtttcagtccctcaggagttacgtcttgtgaagtgatgaacttctggaaggttgcagtgttaactccgctgtattgacgggcatatccgtacgttggcaaagtgtggttggtaccggaggagtaatctccacaactctctggagagtaggcaccaacaaacacagatccagcgtgttgtacttgatcaacataagaagaagcattctcgatttgcaggatcaagtgttcaggagcgtactgattggacatttccaaagcctgctcgtaggttgcaaccgatagggttgtagagtgtgcaatacacttgcgtacaatttcaacccttggcaactgcacagcttggttgtgaacagcatcttcaattctggcaagctccttgtctgtcatatcgacagccaacagaatcacctgggaatcaataccatgttcagcttgagacagaaggtctgaggcaacgaaatctggatcagcgtatttatcagcaataactagaacttcagaaggcccagcaggcatgtcaatactacacagggctgatgtgtcattttgaaccatcatcttggcagcagtaacgaactggtttcctggaccaaatattttgtcacacttaggaacagtttctgttccgtaagccatagcagctactgcctgggcgcctcctgctagcacgatacacttagcaccaaccttgtgggcaacgtagatgacttctggggtaagggtaccatccttcttaggtggagatgcaaaaacaatttctttgcaaccagcaactttggcaggaacacccagcatcagggaagtggaaggcagaattgcggttccaccaggaatatagaggccaactttctcaataggtcttgcaaaacgagagcagactacaccagggcaagtctcaacttgcaacgtctccgttagttgagcttcatggaatttcctgacgttatctatagagagatcaatggctctcttaacgttatctggcaattgcataagttcctctgggaaaggagcttctaacacaggtgtcttcaaagcgactccatcaaacttggcagttagttctaaaagggctttgtcaccattttgacgaacattgtcgacaattggtttgactaattccataatctgttccgttttctggataggacgacgaagggcatcttcaatttcttgtgaggaggccttagaaacgtcaattttgcacaattcaatacgaccttcagaagggacttctttaggtttggattcttctttaggttgttccttggtgtatcctggcttggcatctcctttccttctagtgacctttagggacttcatatccaggtttctctccacctcgtccaacgtcacaccgtacttggcacatctaactaatgcaaaataaaataagtcagcacattcccaggctatatcttccttggatttagcttctgcaagttcatcagcttcctccctaattttagcgttcaacaaaacttcgtcgtcaaataaccgtttggtataagaaccttctggagcattgctcttacgatcccacaaggtggcttccatggctctaagaccctttgattggccaaaacaggaagtgcgttccaagtgacagaaaccaacacctgtttgttcaaccacaaatttcaagcagtctccatcacaatccaattcgatacccagcaacttttgagttgctccagatgtagcacctttataccacaaaccgtgacgacgagattggtagactccagtttgtgtccttatagcctccggaatagactttttggacgagtacaccaggcccaacgagtaattagaagagtcagccaccaaagtagtgaatagaccatcggggcggtcagtagtcaaagacgccaacaaaatttcactgacagggaactttttgacatcttcagaaagttcgtattcagtagtcaattgccgagcatcaataatggggattataccagaagcaacagtggaagtcacatctaccaactttgcggtctcagaaaaagcataaacagttctactaccgccattagtgaaacttttcaaatcgcccagtggagaagaaaaaggcacagcgatactagcattagcgggcaaggatgcaactttatcaaccagggtcctatagataaccctagcgcctgggatcatcctttggacaactctttctgccaaatctaggtccaaaatcacttcattgataccattattgtacaacttgagcaagttgtcgatcagctcctcaaattggtcctctgtaacggatgactcaacttgcacattaacttgaagctcagtcgattgagtgaacttgatcaggttgtgcagctggtcagcagcatagggaaacacggcttttcctaccaaactcaaggaattatcaaactctgcaacacttgcgtatgcaggtagcaagggaaatgtcatacttgaagtcggacagtgagtgtagtcttgagaaattctgaagccgtatttttattatcagtgagtcagtcatcaggagatcctctacgccggacgcatcgtggccggcatcaccggcgccacaggtgcggttgctggcgcctatatcgccgacatcaccgatggggaagatcgggctcgccacttcgggctcatgagcgcttgtttcggcgtgggtatggtggcaggccccgtggccgggggactgttgggcgccatctccttgcatgcaccattccttgcggcggcggtgctcaacggcctcaacctactactgggctgcttcctaatgcaggagtcgcataagggagagcgtcgagtatctatgattggaagtatgggaatggtgatacccgcattcttcagtgtcttgaggtctcctatcagattatgcccaactaaagcaaccggaggaggagatttcatggtaaatttctctgacttttggtcatcagtagactcgaactgtgagactatctcggttatgacagcagaaatgtccttcttggagacagtaaatgaagtcccaccaataaagaaatccttgttatcaggaacaaacttcttgtttcgaactttttcggtgccttgaactataaaatgtagagtggatatgtcgggtaggaatggagcgggcaaatgcttaccttctggaccttcaagaggtatgtagggtttgtagatactgatgccaacttcagtgacaacgttgctatttcgttcaaaccattccgaatccagagaaatcaaagttgtttgtctactattgatccaagccagtgcggtcttgaaactgacaatagtgtgctcgtgttttgaggtcatctttgtatgaataaatctagtctttgatctaaataatcttgacgagccaaggcgataaatacccaaatctaaaactcttttaaaacgttaaaaggacaagtatgtctgcctgtattaaaccccaaatcagctcgtagtctgatcctcatcaacttgaggggcactatcttgttttagagaaatttgcggagatgcgatatcgagaaaaaggtacgctgattttaaacgtgaaatttatctcaagatct

SEQ ID NO: 21 - DNA, 6048 bp, synthetic construct
  source 1..6048: mol_type = other DNA; note = Nucleotide sequence of heterologous nucleic acid molecule comprising a nucleic acid sequence encoding a rabbit myoglobin
aacatccaaagacgaaaggttgaatgaaacctttttgccatccgacatccacaggtccattctcacacataagtgccaaacgcaacaggaggggatacactagcagcagaccgttgcaaacgcaggacctccactcctcttctcctcaacacccacttttgccatcgaaaaaccagcccagttattgggcttgattggagctcgctcattccaattccttctattaggctactaacaccatgactttattagcctgtctatcctggcccccctggcgaggttcatgtttgtttatttccgaatgcaacaagctccgcattacacccgaacatcactccagatgagggctttctgagtgtggggtcaaatagtttcatgttccccaaatggcccaaaactgacagtttaaacgctgtcttggaacctaatatgacaaaagcgtgatctcatccaagatgaactaagtttggttcgttgaaatgctaacggccagttggtcaaaaagaaacttccaaaagtcgccataccgtttgtcttgtttggtattgattgacgaatgctcaaaaataatctcattaatgcttagcgcagtctctctatcgcttctgaaccccggtgcacctgtgccgaaacgcaaatggggaaacacccgctttttggatgattatgcattgtctccacattgtatgcttccaagattctggtgggaatactgctgatagcctaacgttcatgatcaaaatttaactgttctaacccctacttgacagcaatatataaacagaaggaagctgccctgtcttaaacctttttttttatcatcattattagcttactttcataattgcgactggttccaattgacaagcttttgattttaacgacttttaacgacaacttgagaagatcaaaaaacaactaattattcgaaacgatgagattcccatctattttcactgctgttttgttcgctgcttcttctgctttggctgctccagttaacactactactgaagatgagactgctcaaattcctgctgaagctgttattggttactctgatttggagggtgacttcgatgttgctgttttgcctttttctaactctactaacaatggtttgttgttcattaacactactattgcttctattgctgctaaggaagagggtgtttctttggagaaaagagaggctgaagctggtttgtctgacgctgaatggcagcttgttttgaacgtttgggggaaggttgaagctgacctggccggacatggtcaagaggtactcattagactttttcatacgcacccagaaactttagagaagtttgataaatttaaacaccttaagagcgaggatgaaatgaaggcctcggaagatttaaaaaagcacggtaataccgtgctgactgcattgggtgcaattttgaaaaagaagggtcatcacgaagctgaaattaaaccactagctcaatctcatgcaacaaagcataagatccccgtcaagtacttagagttcatctccgaggccattatacatgtcttgcattcaaaacaccctggcgactttggagccgatgctcaggcggcaatgagtaaagctctggaattgttccgtaacgatatcgctgctcaatataaagagctaggattccaaggataagaattaattcgccttagacatgactgttcctcagttcaagttgggcacttacgagaagaccggtcttgctagattctaatcaagaggatgtcagaatgccatttgcctgagagatgcaggcttcatttttgatacttttttatttgtaacctatatagtataggattttttttgtcattttgtttcttctcgtacgagcttgctcctgatcagcctatctcgcagctgatgaatatcttgtggtaggggtttgggaaaatcattcgagtttgatgtttttcttggtatttcccactcctcttcagagtacagaagattaagtgagacgttcgtttgtgcaagcttatcgataagctttaatgcggtagtttatcacagttaaattgctaacgcagtcaggcaccgtgtatgaaatctaacaatgcgctcatcgtcatcctcggcaccgtcaccctggatgctgtaggcataggcttggttatgccggtactgccgggcctcttgcgggatatcgtccattccgacagcatcgccagtcactatggcgtgctgctagcgctatatgcgttgatgcaatttctatgcgcacccgttctcggagcactgtccgaccgctttggccgccgcccagtcctgctcgcttcgctacttggagccactatcgactacgcgatcatggcgaccacacccgtcctgtggatctatcgaatctaaatgtaagttaaaatctctaaataattaaataagtcccagtttctccatacgaaccttaacagcattgcggtgagcatctagaccttcaacagcagccagatccatcactgcttggccaatatgtttcagtccctcaggagttacgtcttgtgaagtgatgaacttctggaaggttgcagtgttaactccgctgtattgacgggcatatccgtacgttggcaaagtgtggttggtaccggaggagtaatctccacaactctctggagagtaggcaccaacaaacacagatccagcgtgttgtacttgatcaacataagaagaagcattctcgatttgcaggatcaagtgttcaggagcgtactgattggacatttccaaagcctgctcgtaggttgcaaccgatagggttgtagagtgtgcaatacacttgcgtacaatttcaacccttggcaactgcacagcttggttgtgaacagcatcttcaattctggcaagctccttgtctgtcatatcgacagccaacagaatcacctgggaatcaataccatgttcagcttgagacagaaggtctgaggcaacgaaatctggatcagcgtatttatcagcaataactagaacttcagaaggcccagcaggcatgtcaatactacacagggctgatgtgtcattttgaaccatcatcttggcagcagtaacgaactggtttcctggaccaaatattttgtcacacttaggaacagtttctgttccgtaagccatagcagctactgcctgggcgcctcctgctagcacgatacacttagcaccaaccttgtgggcaacgtagatgacttctggggtaagggtaccatccttcttaggtggagatgcaaaaacaatttctttgcaaccagcaactttggcaggaacacccagcatcagggaagtggaaggcagaattgcggttccaccaggaatatagaggccaactttctcaataggtcttgcaaaacgagagcagactacaccagggcaagtctcaacttgcaacgtctccgttagttgagcttcatggaatttcctgacgttatctatagagagatcaatggctctcttaacgttatctggcaattgcataagttcctctgggaaaggagcttctaacacaggtgtcttcaaagcgactccatcaaacttggcagttagttctaaaagggctttgtcaccattttgacgaacattgtcgacaattggtttgactaattccataatctgttccgttttctggataggacgacgaagggcatcttcaatttcttgtgaggaggccttagaaacgtcaattttgcacaattcaatacgaccttcagaagggacttctttaggtttggattcttctttaggttgttccttggtgtatcctggcttggcatctcctttccttctagtgacctttagggacttcatatccaggtttctctccacctcgtccaacgtcacaccgtacttggcacatctaactaatgcaaaataaaataagtcagcacattcccaggctatatcttccttggatttagcttctgcaagttcatcagcttcctccctaattttagcgttcaacaaaacttcgtcgtcaaataaccgtttggtataagaaccttctggagcattgctcttacgatcccacaaggtggcttccatggctctaagaccctttgattggccaaaacaggaagtgcgttccaagtgacagaaaccaacacctgtttgttcaaccacaaatttcaagcagtctccatcacaatccaattcgatacccagcaacttttgagttgctccagatgtagcacctttataccacaaaccgtgacgacgagattggtagactccagtttgtgtccttatagcctccggaatagactttttggacgagtacaccaggcccaacgagtaattagaagagtcagccaccaaagtagtgaatagaccatcggggcggtcagtagtcaaagacgccaacaaaatttcactgacagggaactttttgacatcttcagaaagttcgtattcagtagtcaattgccgagcatcaataatggggattataccagaagcaacagtggaagtcacatctaccaactttgcggtctcagaaaaagcataaacagttctactaccgccattagtgaaacttttcaaatcgcccagtggagaagaaaaaggcacagcgatactagcattagcgggcaaggatgcaactttatcaaccagggtcctatagataaccctagcgcctgggatcatcctttggacaactctttctgccaaatctaggtccaaaatcacttcattgataccattattgtacaacttgagcaagttgtcgatcagctcctcaaattggtcctctgtaacggatgactcaacttgcacattaacttgaagctcagtcgattgagtgaacttgatcaggttgtgcagctggtcagcagcatagggaaacacggcttttcctaccaaactcaaggaattatcaaactctgcaacacttgcgtatgcaggtagcaagggaaatgtcatacttgaagtcggacagtgagtgtagtcttgagaaattctgaagccgtatttttattatcagtgagtcagtcatcaggagatcctctacgccggacgcatcgtggccggcatcaccggcgccacaggtgcggttgctggcgcctatatcgccgacatcaccgatggggaagatcgggctcgccacttcgggctcatgagcgcttgtttcggcgtgggtatggtggcaggccccgtggccgggggactgttgggcgccatctccttgcatgcaccattccttgcggcggcggtgctcaacggcctcaacctactactgggctgcttcctaatgcaggagtcgcataagggagagcgtcgagtatctatgattggaagtatgggaatggtgatacccgcattcttcagtgtcttgaggtctcctatcagattatgcccaactaaagcaaccggaggaggagatttcatggtaaatttctctgacttttggtcatcagtagactcgaactgtgagactatctcggttatgacagcagaaatgtccttcttggagacagtaaatgaagtcccaccaataaagaaatccttgttatcaggaacaaacttcttgtttcgaactttttcggtgccttgaactataaaatgtagagtggatatgtcgggtaggaatggagcgggcaaatgcttaccttctggaccttcaagaggtatgtagggtttgtagatactgatgccaacttcagtgacaacgttgctatttcgttcaaaccattccgaatccagagaaatcaaagttgtttgtctactattgatccaagccagtgcggtcttgaaactgacaatagtgtgctcgtgttttgaggtcatctttgtatgaataaatctagtctttgatctaaataatcttgacgagccaaggcgataaatacccaaatctaaaactcttttaaaacgttaaaaggacaagtatgtctgcctgtattaaaccccaaatcagctcgtagtctgatcctcatcaacttgaggggcactatcttgttttagagaaatttgcggagatgcgatatcgagaaaaaggtacgctgattttaaacgtgaaatttatctcaagatct

SEQ ID NO: 22 - DNA, 6048 bp, synthetic construct; identical to SEQ ID NO: 19
  source 1..6048: mol_type = other DNA; note = Nucleotide sequence of heterologous nucleic acid molecule comprising a nucleic acid sequence encoding a bovine myoglobin

SEQ ID NO: 23 - DNA, 6048 bp, synthetic construct
  source 1..6048: mol_type = other DNA; note = Nucleotide sequence of heterologous nucleic acid molecule comprising a nucleic acid sequence encoding a mouse myoglobin
aacatccaaagacgaaaggttgaatgaaacctttttgccatccgacatccacaggtccattctcacacataagtgccaaacgcaacaggaggggatacactagcagcagaccgttgcaaacgcaggacctccactcctcttctcctcaacacccacttttgccatcgaaaaaccagcccagttattgggcttgattggagctcgctcattccaattccttctattaggctactaacaccatgactttattagcctgtctatcctggcccccctggcgaggttcatgtttgtttatttccgaatgcaacaagctccgcattacacccgaacatcactccagatgagggctttctgagtgtggggtcaaatagtttcatgttccccaaatggcccaaaactgacagtttaaacgctgtcttggaacctaatatgacaaaagcgtgatctcatccaagatgaactaagtttggttcgttgaaatgctaacggccagttggtcaaaaagaaacttccaaaagtcgccataccgtttgtcttgtttggtattgattgacgaatgctcaaaaataatctcattaatgcttagcgcagtctctctatcgcttctgaaccccggtgcacctgtgccgaaacgcaaatggggaaacacccgctttttggatgattatgcattgtctccacattgtatgcttccaagattctggtgggaatactgctgatagcctaacgttcatgatcaaaatttaactgttctaacccctacttgacagcaatatataaacagaaggaagctgccctgtcttaaacctttttttttatcatcattattagcttactttcataattgcgactggttccaattgacaagcttttgattttaacgacttttaacgacaacttgagaagatcaaaaaacaactaattattcgaaacgatgagattcccatctattttcactgctgttttgttcgctgcttcttctgctttggctgctccagttaacactactactgaagatgagactgctcaaattcctgctgaagctgttattggttactctgatttggagggtgacttcgatgttgctgttttgcctttttctaactctactaacaatggtttgttgttcattaacactactattgcttctattgctgctaaggaagagggtgtttctttggagaaaagagaggctgaagctggtttgtctgatggagaatggcaacttgttttgaatgtttggggtaaagttgaggctgatcttgctggtcatggtcaagaggttttgattggattgttcaaaactcacccagaaactttggataaattcgataagttcaagaatttgaaaagtgaagaggatatgaagggttctgaggatttgaagaaacacggttgtactgttttgactgctttgggtactattttgaagaaaaaaggtcaacatgctgctgaaattcaaccattggctcaaagtcacgctactaagcacaagattcctgttaagtacttggagttcatttctgagattattattgaagttcttaaaaaaagacattctggtgatttcggtgctgatgctcaaggtgctatgagtaaggctttggaattgttcagaaacgatattgctgctaaatacaaggagcttggttttcaaggttaagaattaattcgccttagacatgactgttcctcagttcaagttgggcacttacgagaagaccggtcttgctagattctaatcaagaggatgtcagaatgccatttgcctgagagatgcaggcttcatttttgatacttttttatttgtaacctatatagtataggattttttttgtcattttgtttcttctcgtacgagcttgctcctgatcagcctatctcgcagctgatgaatatcttgtggtaggggtttgggaaaatcattcgagtttgatgtttttcttggtatttcccactcctcttcagagtacagaagattaagtgagacgttcgtttgtgcaagcttatcgataagctttaatgcggtagtttatcacagttaaattgctaacgcagtcaggcaccgtgtatgaaatctaacaatgcgctcatcgtcatcctcggcaccgtcaccctggatgctgtaggcataggcttggttatgccggtactgccgggcctcttgcgggatatcgtccattccgacagcatcgccagtcactatggcgtgctgctagcgctatatgcgttgatgcaatttctatgcgcacccgttctcggagcactgtccgaccgctttggccgccgcccagtcctgctcgcttcgctacttggagccactatcgactacgcgatcatggcgaccacacccgtcctgtggatctatcgaatctaaatgtaagttaaaatctctaaataattaaataagtcccagtttctccatacgaaccttaacagcattgcggtgagcatctagaccttcaacagcagccagatccatcactgcttggccaatatgtttcagtccctcaggagttacgtcttgtgaagtgatgaacttctggaaggttgcagtgttaactccgctgtattgacgggcatatccgtacgttggcaaagtgtggttggtaccggaggagtaatctccacaactctctggagagtaggcaccaacaaacacagatccagcgtgttgtacttgatcaacataagaagaagcattctcgatttgcaggatcaagtgttcaggagcgtactgattggacatttccaaagcctgctcgtaggttgcaaccgatagggttgtagagtgtgcaatacacttgcgtacaatttcaacccttggcaactgcacagcttggttgtgaacagcatcttcaattctggcaagctccttgtctgtcatatcgacagccaacagaatcacctgggaatcaataccatgttcagcttgagacagaaggtctgaggcaacgaaatctggatcagcgtatttatcagcaataactagaacttcagaaggcccagcaggcatgtcaatactacacagggctgatgtgtcattttgaaccatcatcttggcagcagtaacgaactggtttcctggaccaaatattttgtcacacttaggaacagtttctgttccgtaagccatagcagctactgcctgggcgcctcctgctagcacgatacacttagcaccaaccttgtgggcaacgtagatgacttctggggtaagggtaccatccttcttaggtggagatgcaaaaacaatttctttgcaaccagcaactttggcaggaacacccagcatcagggaagtggaaggcagaattgcggttccaccaggaatatagaggccaactttctcaataggtcttgcaaaacgagagcagactacaccagggcaagtctcaacttgcaacgtctccgttagttgagcttcatggaatttcctgacgttatctatagagagatcaatggctctcttaacgttatctggcaattgcataagttcctctgggaaaggagcttctaacacaggtgtcttcaaagcgactccatcaaacttggcagttagttctaaaagggctttgtcaccattttgacgaacattgtcgacaattggtttgactaattccataatctgttccgttttctggataggacgacgaagggcatcttcaatttcttgtgaggaggccttagaaacgtcaattttgcacaattcaatacgaccttcagaagggacttctttaggtttggattcttctttaggttgttccttggtgtatcctggcttggcatctcctttccttctagtgacctttagggacttcatatccaggtttctctccacctcgtccaacgtcacaccgtacttggcacatctaactaatgcaaaataaaataagtcagcacattcccaggctatatcttccttggatttagcttctgcaagttcatcagcttcctccctaattttagcgttcaacaaaacttcgtcgtcaaataaccgtttggtataagaaccttctggagcattgctcttacgatcccacaaggtggcttccatggctctaagaccctttgattggccaaaacaggaagtgcgttccaagtgacagaaaccaacacctgtttgttcaaccacaaatttcaagcagtctccatcacaatccaattcgatacccagcaacttttgagttgctccagatgtagcacctttataccacaaaccgtgacgacgagattggtagactccagtttgtgtccttatagcctccggaatagactttttggacgagtacaccaggcccaacgagtaattagaagagtcagccaccaaagtagtgaatagaccatcggggcggtcagtagtcaaagacgccaacaaaatttcactgacagggaactttttgacatcttcagaaagttcgtattcagtagtcaattgccgagcatcaataatggggattataccagaagcaacagtggaagtcacatctaccaactttgcggtctcagaaaaagcataaacagttctactaccgccattagtgaaacttttcaaatcgcccagtggagaagaaaaaggcacagcgatactagcattagcgggcaaggatgcaactttatcaaccagggtcctatagataaccctagcgcctgggatcatcctttggacaactctttctgccaaatctaggtccaaaatcacttcattgataccattattgtacaacttgagcaagttgtcgatcagctcctcaaattggtcctctgtaacggatgactcaacttgcacattaacttgaagctcagtcgattgagtgaacttgatcaggttgtgcagctggtcagcagcatagggaaacacggcttttcctaccaaactcaaggaattatcaaactctgcaacacttgcgtatgcaggtagcaagggaaatgtcatacttgaagtcggacagtgagtgtagtcttgagaaattctgaagccgtatttttattatcagtgagtcagtcatcaggagatcctctacgccggacgcatcgtggccggcatcaccggcgccacaggtgcggttgctggcgcctatatcgccgacatcaccgatggggaagatcgggctcgccacttcgggctcatgagcgcttgtttcggcgtgggtatggtggcaggccccgtggccgggggactgttgggcgccatctccttgcatgcaccattccttgcggcggcggtgctcaacggcctcaacctactactgggctgcttcctaatgcaggagtcgcataagggagagcgtcgagtatctatgattggaagtatgggaatggtgatacccgcattcttcagtgtcttgaggtctcctatcagattatgcccaactaaagcaaccggaggaggagatttcatggtaaatttctctgacttttggtcatcagtagactcgaactgtgagactatctcggttatgacagcagaaatgtccttcttggagacagtaaatgaagtcccaccaataaagaaatccttgttatcaggaacaaacttcttgtttcgaactttttcggtgccttgaactataaaatgtagagtggatatgtcgggtaggaatggagcgggcaaatgcttaccttctggaccttcaagaggtatgtagggtttgtagatactgatgccaacttcagtgacaacgttgctatttcgttcaaaccattccgaatccagagaaatcaaagttgtttgtctactattgatccaagccagtgcggtcttgaaactgacaatagtgtgctcgtgttttgaggtcatctttgtatgaataaatctagtctttgatctaaataatcttgacgagccaaggcgataaatacccaaatctaaaactcttttaaaacgttaaaaggacaagtatgtctgcctgtattaaaccccaaatcagctcgtagtctgatcctcatcaacttgaggggcactatcttgttttagagaaatttgcggagatgcgatatcgagaaaaaggtacgctgattttaaacgtgaaatttatctcaagatct

SEQ ID NO: 24 - DNA, 6048 bp, synthetic construct
  source 1..6048: mol_type = other DNA; note = Nucleotide sequence of heterologous nucleic acid molecule comprising a nucleic acid sequence encoding a rat myoglobin
aacatccaaagacgaaaggttgaatgaaacctttttgccatccgacatccacaggtccattctcacacataagtgccaaacgcaacaggaggggatacactagcagcagaccgttgcaaacgcaggacctccactcctcttctcctcaacacccacttttgccatcgaaaaaccagcccagttattgggcttgattggagctcgctcattccaattccttctattaggctactaacaccatgactttattagcctgtctatcctggcccccctggcgaggttcatgtttgtttatttccgaatgcaacaagctccgcattacacccgaacatcactccagatgagggctttctgagtgtggggtcaaatagtttcatgttccccaaatggcccaaaactgacagtttaaacgctgtcttggaacctaatatgacaaaagcgtgatctcatccaagatgaactaagtttggttcgttgaaatgctaacggccagttggtcaaaaagaaacttccaaaagtcgccataccgtttgtcttgtttggtattgattgacgaatgctcaaaaataatctcattaatgcttagcgcagtctctctatcgcttctgaaccccggtgcacctgtgccgaaacgcaaatggggaaacacccgctttttggatgattatgcattgtctccacattgtatgcttccaagattctggtgggaatactgctgatagcctaacgttcatgatcaaaatttaactgttctaacccctacttgacagcaatatataaacagaaggaagctgccctgtcttaaacctttttttttatcatcattattagcttactttcataattgcgactggttccaattgacaagcttttgattttaacgacttttaacgacaacttgagaagatcaaaaaacaactaattattcgaaacgatgagattcccatctattttcactgctgttttgttcgctgcttcttctgctttggctgctccagttaacactactactgaagatgagactgctcaaattcctgctgaagctgttattggttactctgatttggagggtgacttcgatgttgctgttttgcctttttctaactctactaacaatggtttgttgttcattaacactactattgcttctattgctgctaaggaagagggtgtttctttggagaaaagagaggctgaagctggtctctccgatggagaatggcaaatggttcttaatatatggggcaaagtggaaggtgacctagcaggtcacggacaagaagttctgatctctttattcaaggcacatccagagacgttagaaaagttcgataaatttaagaacttgaagtcggaagaagaaatgaagtcatccgaggatctgaaaaagcacggatgtactgtccttacagcattgggaactatcttgaaaaagaaaggtcaacacgctgctgagattcagcccttggcccaaagccatgctaccaaacataagattcctgtcaagtacttagaatttatttctgaggttattatacaggtactgaaaaaacgttacagtggagacttcggtgctgacgcccaaggtgctatgtcaaaagctttggagctttttagaaacgatatcgccgcgaagtataaggagctaggctttcaggggtaagaattaattcgccttagacatgactgttcctcagttcaagttgggcacttacgagaagaccggtcttgctagattctaatcaagaggatgtcagaatgccatttgcctgagagatgcaggcttcatttttgatacttttttatttgtaacctatatagtataggattttttttgtcattttgtttcttctcgtacgagcttgctcctgatcagcctatctcgcagctgatgaatatcttgtggtaggggtttgggaaaatcattcgagtttgatgtttttcttggtatttcccactcctcttcagagtacagaagattaagtgagacgttcgtttgtgcaagcttatcgataagctttaatgcggtagtttatcacagttaaattgctaacgcagtcaggcaccgtgtatgaaatctaacaatgcgctcatcgtcatcctcggcaccgtcaccctggatgctgtaggcataggcttggttatgccggtactgccgggcctcttgcgggatatcgtccattccgacagcatcgccagtcactatggcgtgctgctagcgctatatgcgttgatgcaatttctatgcgcacccgttctcggagcactgtccgaccgctttggccgccgcccagtcctgctcgcttcgctacttggagccactatcgactacgcgatcatggcgaccacacccgtcctgtggatctatcgaatctaaatgtaagttaaaatctctaaataattaaataagtcccagtttctccatacgaaccttaacagcattgcggtgagcatctagaccttcaacagcagccagatccatcactgcttggccaatatgtttcagtccctcaggagttacgtcttgtgaagtgatgaacttctggaaggttgcagtgttaactccgctgtattgacgggcatatccgtacgttggcaaagtgtggttggtaccggaggagtaatctccacaactctctggagagtaggcaccaacaaacacagatccagcgtgttgtacttgatcaacataagaagaagcattctcgatttgcaggatcaagtgttcaggagcgtactgattggacatttccaaagcctgctcgtaggttgcaaccgatagggttgtagagtgtgcaatacacttgcgtacaatttcaacccttggcaactgcacagcttggttgtgaacagcatcttcaattctggcaagctccttgtctgtcatatcgacagccaacagaatcacctgggaatcaataccatgttcagcttgagacagaaggtctgaggcaacgaaatctggatcagcgtatttatcagcaataactagaacttcagaaggcccagcaggcatgtcaatactacacagggctgatgtgtcattttgaaccatcatcttggcagcagtaacgaactggtttcctggaccaaatattttgtcacacttaggaacagtttctgttccgtaagccatagcagctactgcctgggcgcctcctgctagcacgatacacttagcaccaaccttgtgggcaacgtagatgacttctggggtaagggtaccatccttcttaggtggagatgcaaaaacaatttctttgcaaccagcaactttggcaggaacacccagcatcagggaagtggaaggcagaattgcggttccaccaggaatatagaggccaactttctcaataggtcttgcaaaacgagagcagactacaccagggcaagtctcaacttgcaacgtctccgttagttgagcttcatggaatttcctgacgttatctatagagagatcaatggctctcttaacgttatctggcaattgcataagttcctctgggaaaggagcttctaacacaggtgtcttcaaagcgactccatcaaacttggcagttagttctaaaagggctttgtcaccattttgacgaacattgtcgacaattggtttgactaattccataatctgttccgttttctggataggacgacgaagggcatcttcaatttcttgtgaggaggccttagaaacgtcaattttgcacaattcaatacgaccttcagaagggacttctttaggtttggattcttctttaggttgttccttggtgtatcctggcttggcatctcctttccttctagtgacctttagggacttcatatccaggtttctctccacctcgtccaacgtcacaccgtacttggcacatctaactaatgcaaaataaaataagtcagcacattcccaggctatatcttccttggatttagcttctgcaagttcatcagcttcctccctaattttagcgttcaacaaaacttcgtcgtcaaataaccgtttggtataagaaccttctggagcattgctcttacgatcccacaaggtggcttccatggctctaagaccctttgattggccaaaacaggaagtgcgttccaagtgacagaaaccaacacctgtttgttcaaccacaaatttcaagcagtctccatcacaatccaattcgatacccagcaacttttgagttgctccagatgtagcacctttataccacaaaccgtgacgacgagattggtagactccagtttgtgtccttatagcctccggaatagactttttggacgagtacaccaggcccaacgagtaattagaagagtcagccaccaaagtagtgaatagaccatcggggcggtcagtagtcaaagacgccaacaaaatttcactgacagggaactttttgacatcttcagaaagttcgtattcagtagtcaattgccgagcatcaataatggggattataccagaagcaacagtggaagtcacatctaccaactttgcggtctcagaaaaagcataaacagttctactaccgccattagtgaaacttttcaaatcgcccagtggagaagaaaaaggcacagcgatactagcattagcgggcaaggatgcaactttatcaaccagggtcctatagataaccctagcgcctgggatcatcctttggacaactctttctgccaaatctaggtccaaaatcacttcattgataccattattgtacaacttgagcaagttgtcgatcagctcctcaaattggtcctctgtaacggatgactcaacttgcacattaacttgaagctcagtcgattgagtgaacttgatcaggttgtgcagctggtcagcagcatagggaaacacggcttttcctaccaaactcaaggaattatcaaactctgcaacacttgcgtatgcaggtagcaagggaaatgtcatacttgaagtcggacagtgagtgtagtcttgagaaattctgaagccgtatttttattatcagtgagtcagtcatcaggagatcctctacgccggacgcatcgtggccggcatcaccggcgccacaggtgcggttgctggcgcctatatcgccgacatcaccgatggggaagatcgggctcgccacttcgggctcatgagcgcttgtttcggcgtgggtatggtggcaggccccgtggccgggggactgttgggcgccatctccttgcatgcaccattccttgcggcggcggtgctcaacggcctcaacctactactgggctgcttcctaatgcaggagtcgcataagggagagcgtcgagtatctatgattggaagtatgggaatggtgatacccgcattcttcagtgtcttgaggtctcctatcagattatgcccaactaaagcaaccggaggaggagatttcatggtaaatttctctgacttttggtcatcagtagactcgaactgtgagactatctcggttatgacagcagaaatgtccttcttggagacagtaaatgaagtcccaccaataaagaaatccttgttatcaggaacaaacttcttgtttcgaactttttcggtgccttgaactataaaatgtagagtggatatgtcgggtaggaatggagcgggcaaatgcttaccttctggaccttcaagaggtatgtagggtttgtagatactgatgccaacttcagtgacaacgttgctatttcgttcaaaccattccgaatccagagaaatcaaagttgtttgtctactattgatccaagccagtgcggtcttgaaactgacaatagtgtgctcgtgttttgaggtcatctttgtatgaataaatctagtctttgatctaaataatcttgacgagccaaggcgataaatacccaaatctaaaactcttttaaaacgttaaaaggacaagtatgtctgcctgtattaaaccccaaatcagctcgtagtctgatcctcatcaacttgaggggcactatcttgttttagagaaatttgcggagatgcgatatcgagaaaaaggtacgctgattttaaacgtgaaatttatctcaagatct

SEQ ID NO: 25 - DNA, 6027 bp, synthetic construct
  source 1..6027: mol_type = other DNA; note = Nucleotide sequence of heterologous nucleic acid molecule comprising a nucleic acid sequence encoding a tuna myoglobin
aacatccaaagacgaaaggttgaatgaaacctttttgccatccgacatccacaggtccattctcacacataagtgccaaacgcaacaggaggggatacactagcagcagaccgttgcaaacgcaggacctccactcctcttctcctcaacacccacttttgccatcgaaaaaccagcccagttattgggcttgattggagctcgctcattccaattccttctattaggctactaacaccatgactttattagcctgtctatcctggcccccctggcgaggttcatgtttgtttatttccgaatgcaacaagctccgcattacacccgaacatcactccagatgagggctttctgagtgtggggtcaaatagtttcatgttccccaaatggcccaaaactgacagtttaaacgctgtcttggaacctaatatgacaaaagcgtgatctcatccaagatgaactaagtttggttcgttgaaatgctaacggccagttggtcaaaaagaaacttccaaaagtcgccataccgtttgtcttgtttggtattgattgacgaatgctcaaaaataatctcattaatgcttagcgcagtctctctatcgcttctgaaccccggtgcacctgtgccgaaacgcaaatggggaaacacccgctttttggatgattatgcattgtctccacattgtatgcttccaagattctggtgggaatactgctgatagcctaacgttcatgatcaaaatttaactgttctaacccctacttgacagcaatatataaacagaaggaagctgccctgtcttaaacctttttttttatcatcattattagcttactttcataattgcgactggttccaattgacaagcttttgattttaacgacttttaacgacaacttgagaagatcaaaaaacaactaattattcgaaacgatgagattcccttctattttcactgctgttttgtttgctgcttcttctgctttggctgctccagttaacactactactgaagatgagactgctcaaattccagctgaagctgttattggttactctgatttggagggtgacttcgatgttgctgttttgccattctctaactctactaataacggtttgttgtttattaacactactattgcttctattgctgctaaggaggaaggtgtttctttggagaaaagagaagctgaggctgctgatttcgatgctgttttgaagtgttggggtccagttgaagctgattacactactattggtggtttggttttgactagattgttcaaggagcatccagaaactcaaaagttgtttccaaagttcgctggtattgctcaagctgatattgctggtaacgctgctgtttctgctcatggtgctactgttttgaagaaattgggtgaattgttgaaggctaaaggttctcatgctgctattttgaagccattggctaactctcacgctactaaacacaagattccaattaacaatttcaagttgatttctgaggttttggttaaggttatgcacgaaaaggctggtttggatgctggtggtcaaactgctttgagaaacgttatgggtattattattgctgatttggaagctaactacaaggaattgggtttttctggttaagaattaattcgccttagacatgactgttcctcagttcaagttgggcacttacgagaagaccggtcttgctagattctaatcaagaggatgtcagaatgccatttgcctgagagatgcaggcttcatttttgatacttttttatttgtaacctatatagtataggattttttttgtcattttgtttcttctcgtacgagcttgctcctgatcagcctatctcgcagctgatgaatatcttgtggtaggggtttgggaaaatcattcgagtttgatgtttttcttggtatttcccactcctcttcagagtacagaagattaagtgagacgttcgtttgtgcaagcttatcgataagctttaatgcggtagtttatcacagttaaattgctaacgcagtcaggcaccgtgtatgaaatctaacaatgcgctcatcgtcatcctcggcaccgtcaccctggatgctgtaggcataggcttggttatgccggtactgccgggcctcttgcgggatatcgtccattccgacagcatcgccagtcactatggcgtgctgctagcgctatatgcgttgatgcaatttctatgcgcacccgttctcggagcactgtccgaccgctttggccgccgcccagtcctgctcgcttcgctacttggagccactatcgactacgcgatcatggcgaccacacccgtcctgtggatctatcgaatctaaatgtaagttaaaatctctaaataattaaataagtcccagtttctccatacgaaccttaacagcattgcggtgagcatctagaccttcaacagcagccagatccatcactgcttggccaatatgtttcagtccctcaggagttacgtcttgtgaagtgatgaacttctggaaggttgcagtgttaactccgctgtattgacgggcatatccgtacgttggcaaagtgtggttggtaccggaggagtaatctccacaactctctggagagtaggcaccaacaaacacagatccagcgtgttgtacttgatcaacataagaagaagcattctcgatttgcaggatcaagtgttcaggagcgtactgattggacatttccaaagcctgctcgtaggttgcaaccgatagggttgtagagtgtgcaatacacttgcgtacaatttcaacccttggcaactgcacagcttggttgtgaacagcatcttcaattctggcaagctccttgtctgtcatatcgacagccaacagaatcacctgggaatcaataccatgttcagcttgagacagaaggtctgaggcaacgaaatctggatcagcgtatttatcagcaataactagaacttcagaaggcccagcaggcatgtcaatactacacagggctgatgtgtcattttgaaccatcatcttggcagcagtaacgaactggtttcctggaccaaatattttgtcacacttaggaacagtttctgttccgtaagccatagcagctactgcctgggcgcctcctgctagcacgatacacttagcaccaaccttgtgggcaacgtagatgacttctggggtaagggtaccatccttcttaggtggagatgcaaaaacaatttctttgcaaccagcaactttggcaggaacacccagcatcagggaagtggaaggcagaattgcggttccaccaggaatatagaggccaactttctcaataggtcttgcaaaacgagagcagactacaccagggcaagtctcaacttgcaacgtctccgttagttgagcttcatggaatttcctgacgttatctatagagagatcaatggctctcttaacgttatctggcaattgcataagttcctctgggaaaggagcttctaacacaggtgtcttcaaagcgactccatcaaacttggcagttagttctaaaagggctttgtcaccattttgacgaacattgtcgacaattggtttgactaattccataatctgttccgttttctggataggacgacgaagggcatcttcaatttcttgtgaggaggccttagaaacgtcaattttgcacaattcaatacgaccttcagaagggacttctttaggtttggattcttctttaggttgttccttggtgtatcctggcttggcatctcctttccttctagtgacctttagggacttcatatccaggtttctctccacctcgtccaacgtcacaccgtacttggcacatctaactaatgcaaaataaaataagtcagcacattcccaggctatatcttccttggatttagcttctgcaagttcatcagcttcctccctaattttagcgttcaacaaaacttcgtcgtcaaataaccgtttggtataagaaccttctggagcattgctcttacgatcccacaaggtggcttccatggctctaagaccctttgattggccaaaacaggaagtgcgttccaagtgacagaaaccaacacctgtttgttcaaccacaaatttcaagcagtctccatcacaatccaattcgatacccagcaacttttgagttgctccagatgtagcacctttataccacaaaccgtgacgacgagattggtagactccagtttgtgtccttatagcctccggaatagactttttggacgagtacaccaggcccaacgagtaattagaagagtcagccaccaaagtagtgaatagaccatcggggcggtcagtagtcaaagacgccaacaaaatttcactgacagggaactttttgacatcttcagaaagttcgtattcagtagtcaattgccgagcatcaataatggggattataccagaagcaacagtggaagtcacatctaccaactttgcggtctcagaaaaagcataaacagttctactaccgccattagtgaaacttttcaaatcgcccagtggagaagaaaaaggcacagcgatactagcattagcgggcaaggatgcaactttatcaaccagggtcctatagataaccctagcgcctgggatcatcctttggacaactctttctgccaaatctaggtccaaaatcacttcattgataccattattgtacaacttgagcaagttgtcgatcagctcctcaaattggtcctctgtaacggatgactcaacttgcacattaacttgaagctcagtcgattgagtgaacttgatcaggttgtgcagctggtcagcagcatagggaaacacggcttttcctaccaaactcaaggaattatcaaactctgcaacacttgcgtatgcaggtagcaagggaaatgtcatacttgaagtcggacagtgagtgtagtcttgagaaattctgaagccgtatttttattatcagtgagtcagtcatcaggagatcctctacgccggacgcatcgtggccggcatcaccggcgccacaggtgcggttgctggcgcctatatcgccgacatcaccgatggggaagatcgggctcgccacttcgggctcatgagcgcttgtttcggcgtgggtatggtggcaggccccgtggccgggggactgttgggcgccatctccttgcatgcaccattccttgcggcggcggtgctcaacggcctcaacctactactgggctgcttcctaatgcaggagtcgcataagggagagcgtcgagtatctatgattggaagtatgggaatggtgatacccgcattcttcagtgtcttgaggtctcctatcagattatgcccaactaaagcaaccggaggaggagatttcatggtaaatttctctgacttttggtcatcagtagactcgaactgtgagactatctcggttatgacagcagaaatgtccttcttggagacagtaaatgaagtcccaccaataaagaaatccttgttatcaggaacaaacttcttgtttcgaactttttcggtgccttgaactataaaatgtagagtggatatgtcgggtaggaatggagcgggcaaatgcttaccttctggaccttcaagaggtatgtagggtttgtagatactgatgccaacttcagtgacaacgttgctatttcgttcaaaccattccgaatccagagaaatcaaagttgtttgtctactattgatccaagccagtgcggtcttgaaactgacaatagtgtgctcgtgttttgaggtcatctttgtatgaataaatctagtctttgatctaaataatcttgacgagccaaggcgataaatacccaaatctaaaactcttttaaaacgttaaaaggacaagtatgtctgcctgtattaaaccccaaatcagctcgtagtctgatcctcatcaacttgaggggcactatcttgttttagagaaatttgcggagatgcgatatcgagaaaaaggtacgctgattttaaacgtgaaatttatctcaagatct

SEQ ID NO: 26 - DNA, 6027 bp, synthetic construct
  source 1..6027: mol_type = other DNA; note = Nucleotide sequence of heterologous nucleic acid molecule comprising a nucleic acid sequence encoding a salmon myoglobin
aacatccaaagacgaaaggttgaatgaaacctttttgccatccgacatccacaggtccattctcacacataagtgccaaacgcaacaggaggggatacactagcagcagaccgttgcaaacgcaggacctccactcctcttctcctcaacacccacttttgccatcgaaaaaccagcccagttattgggcttgattggagctcgctcattccaattccttctattaggctactaacaccatgactttattagcctgtctatcctggcccccctggcgaggttcatgtttgtttatttccgaatgcaacaagctccgcattacacccgaacatcactccagatgagggctttctgagtgtggggtcaaatagtttcatgttccccaaatggcccaaaactgacagtttaaacgctgtcttggaacctaatatgacaaaagcgtgatctcatccaagatgaactaagtttggttcgttgaaatgctaacggccagttggtcaaaaagaaacttccaaaagtcgccataccgtttgtcttgtttggtattgattgacgaatgctcaaaaataatctcattaatgcttagcgcagtctctctatcgcttctgaaccccggtgcacctgtgccgaaacgcaaatggggaaacacccgctttttggatgattatgcattgtctccacattgtatgcttccaagattctggtgggaatactgctgatagcctaacgttcatgatcaaaatttaactgttctaacccctacttgacagcaatatataaacagaaggaagctgccctgtcttaaacctttttttttatcatcattattagcttactttcataattgcgactggttccaattgacaagcttttgattttaacgacttttaacgacaacttgagaagatcaaaaaacaactaattattcgaaacgatgagattcccatctattttcactgctgttttgttcgctgcttcttctgctttggctgctccagttaacactactactgaggatgaaactgctcaaattccagctgaagctgttattggttactctgatttggagggtgacttcgatgttgctgttttgccattctctaactctactaacaatggtttgttgttcattaacactactattgcttctattgctgctaaggaggaaggtgtttctttggagaagagagaagctgaggctgcaaactacgacatggtcctacaatgttgggagcccgtagaagcagactataataaccacggagggttggtcttgtccagactatttgctgaacatcctgagacgttaacattattcccaaagttcgccggtattgctgcaggtgacctgtctggtaatgctgccgttgccgctcatggcgctactgttttgagaaaattgggagaattacttaacgctaggggtgatcatgccgcgaccctgaaatcactggcaactactcacgcaaacaaacacaagataccattgaagaactttacactcattactaatatcatctgcaaagtgatgggagaaaaggctggtttggatgaagctggtcaagaggcccttcgtcaggtgatgggcgttatcattgctgatattaatgttacctacatggagcttggatttgccggatgagaattaattcgccttagacatgactgttcctcagttcaagttgggcacttacgagaagaccggtcttgctagattctaatcaagaggatgtcagaatgccatttgcctgagagatgcaggcttcatttttgatacttttttatttgtaacctatatagtataggattttttttgtcattttgtttcttctcgtacgagcttgctcctgatcagcctatctcgcagctgatgaatatcttgtggtaggggtttgggaaaatcattcgagtttgatgtttttcttggtatttcccactcctcttcagagtacagaagattaagtgagacgttcgtttgtgcaagcttatcgataagctttaatgcggtagtttatcacagttaaattgctaacgcagtcaggcaccgtgtatgaaatctaacaatgcgctcatcgtcatcctcggcaccgtcaccctggatgctgtaggcataggcttggttatgccggtactgccgggcctcttgcgggatatcgtccattccgacagcatcgccagtcactatggcgtgctgctagcgctatatgcgttgatgcaatttctatgcgcacccgttctcggagcactgtccgaccgctttggccgccgcccagtcctgctcgcttcgctacttggagccactatcgactacgcgatcatggcgaccacacccgtcctgtggatctatcgaatctaaatgtaagttaaaatctctaaataattaaataagtcccagtttctccatacgaaccttaacagcattgcggtgagcatctagaccttcaacagcagccagatccatcactgcttggccaatatgtttcagtccctcaggagttacgtcttgtgaagtgatgaacttctggaaggttgcagtgttaactccgctgtattgacgggcatatccgtacgttggcaaagtgtggttggtaccggaggagtaatctccacaactctctggagagtaggcaccaacaaacacagatccagcgtgttgtacttgatcaacataagaagaagcattctcgatttgcaggatcaagtgttcaggagcgtactgattggacatttccaaagcctgctcgtaggttgcaaccgatagggttgtagagtgtgcaatacacttgcgtacaatttcaacccttggcaactgcacagcttggttgtgaacagcatcttcaattctggcaagctccttgtctgtcatatcgacagccaacagaatcacctgggaatcaataccatgttcagcttgagacagaaggtctgaggcaacgaaatctggatcagcgtatttatcagcaataactagaacttcagaaggcccagcaggcatgtcaatactacacagggctgatgtgtcattttgaaccatcatcttggcagcagtaacgaactggtttcctggaccaaatattttgtcacacttaggaacagtttctgttccgtaagccatagcagctactgcctgggcgcctcctgctagcacgatacacttagcaccaaccttgtgggcaacgtagatgacttctggggtaagggtaccatccttcttaggtggagatgcaaaaacaatttctttgcaaccagcaactttggcaggaacacccagcatcagggaagtggaaggcagaattgcggttccaccaggaatatagaggccaactttctcaataggtcttgcaaaacgagagcagactacaccagggcaagtctcaacttgcaacgtctccgttagttgagcttcatggaatttcctgacgttatctatagagagatcaatggctctcttaacgttatctggcaattgcataagttcctctgggaaaggagcttctaacacaggtgtcttcaaagcgactccatcaaacttggcagttagttctaaaagggctttgtcaccattttgacgaacattgtcgacaattggtttgactaattccataatctgttccgttttctggataggacgacgaagggcatcttcaatttcttgtgaggaggccttagaaacgtcaattttgcacaattcaatacgaccttcagaagggacttctttaggtttggattcttctttaggttgttccttggtgtatcctggcttggcatctcctttccttctagtgacctttagggacttcatatccaggtttctctccacctcgtccaacgtcacaccgtacttggcacatctaactaatgcaaaataaaataagtcagcacattcccaggctatatcttccttggatttagcttctgcaagttcatcagcttcctccctaattttagcgttcaacaaaacttcgtcgtcaaataaccgtttggtataagaaccttctggagcattgctcttacgatcccacaaggtggcttccatggctctaagaccctttgattggccaaaacaggaagtgcgttccaagtgacagaaaccaacacctgtttgttcaaccacaaatttcaagcagtctccatcacaatccaattcgatacccagcaacttttgagttgctccagatgtagcacctttataccacaaaccgtgacgacgagattggtagactccagtttgtgtccttatagcctccggaatagactttttggacgagtacaccaggcccaacgagtaattagaagagtcagccaccaaagtagtgaatagaccatcggggcggtcagtagtcaaagacgccaacaaaatttcactgacagggaactttttgacatcttcagaaagttcgtattcagtagtcaattgccgagcatcaataatggggattataccagaagcaacagtggaagtcacatctaccaactttgcggtctcagaaaaagcataaacagttctactaccgccattagtgaaacttttcaaatcgcccagtggagaagaaaaaggcacagcgatactagcattagcgggcaaggatgcaactttatcaaccagggtcctatagataaccctagcgcctgggatcatcctttggacaactctttctgccaaatctaggtccaaaatcacttcattgataccattattgtacaacttgagcaagttgtcgatcagctcctcaaattggtcctctgtaacggatgactcaacttgcacattaacttgaagctcagtcgattgagtgaacttgatcaggttgtgcagctggtcagcagcatagggaaacacggcttttcctaccaaactcaaggaattatcaaactctgcaacacttgcgtatgcaggtagcaagggaaatgtcatacttgaagtcggacagtgagtgtagtcttgagaaattctgaagccgtatttttattatcagtgagtcagtcatcaggagatcctctacgccggacgcatcgtggccggcatcaccggcgccacaggtgcggttgctggcgcctatatcgccgacatcaccgatggggaagatcgggctcgccacttcgggctcatgagcgcttgtttcggcgtgggtatggtggcaggccccgtggccgggggactgttgggcgccatctccttgcatgcaccattccttgcggcggcggtgctcaacggcctcaacctactactgggctgcttcctaatgcaggagtcgcataagggagagcgtcgagtatctatgattggaagtatgggaatggtgatacccgcattcttcagtgtcttgaggtctcctatcagattatgcccaactaaagcaaccggaggaggagatttcatggtaaatttctctgacttttggtcatcagtagactcgaactgtgagactatctcggttatgacagcagaaatgtccttcttggagacagtaaatgaagtcccaccaataaagaaatccttgttatcaggaacaaacttcttgtttcgaactttttcggtgccttgaactataaaatgtagagtggatatgtcgggtaggaatggagcgggcaaatgcttaccttctggaccttcaagaggtatgtagggtttgtagatactgatgccaacttcagtgacaacgttgctatttcgttcaaaccattccgaatccagagaaatcaaagttgtttgtctactattgatccaagccagtgcggtcttgaaactgacaatagtgtgctcgtgttttgaggtcatctttgtatgaataaatctagtctttgatctaaataatcttgacgagccaaggcgataaatacccaaatctaaaactcttttaaaacgttaaaaggacaagtatgtctgcctgtattaaaccccaaatcagctcgtagtctgatcctcatcaacttgaggggcactatcttgttttagagaaatttgcggagatgcgatatcgagaaaaaggtacgctgattttaaacgtgaaatttatctcaagatct

SEQ ID NO: 27 - DNA, 6027 bp, synthetic construct
  source 1..6027: mol_type = other DNA; note = Nucleotide sequence of heterologous nucleic acid molecule comprising a nucleic acid sequence encoding a Blue bonito myoglobin
aacatccaaagacgaaaggttgaatgaaacctttttgccatccgacatccacaggtccattctcacacataagtgccaaacgcaacaggaggggatacactagcagcagaccgttgcaaacgcaggacctccactcctcttctcctcaacacccacttttgccatcgaaaaaccagcccagttattgggcttgattggagctcgctcattccaattccttctattaggctactaacaccatgactttattagcctgtctatcctggcccccctggcgaggttcatgtttgtttatttccgaatgcaacaagctccgcattacacccgaacatcactccagatgagggctttctgagtgtggggtcaaatagtttcatgttccccaaatggcccaaaactgacagtttaaacgctgtcttggaacctaatatgacaaaagcgtgatctcatccaagatgaactaagtttggttcgttgaaatgctaacggccagttggtcaaaaagaaacttccaaaagtcgccataccgtttgtcttgtttggtattgattgacgaatgctcaaaaataatctcattaatgcttagcgcagtctctctatcgcttctgaaccccggtgcacctgtgccgaaacgcaaatggggaaacacccgctttttggatgattatgcattgtctccacattgtatgcttccaagattctggtgggaatactgctgatagcctaacgttcatgatcaaaatttaactgttctaacccctacttgacagcaatatataaacagaaggaagctgccctgtcttaaacctttttttttatcatcattattagcttactttcataattgcgactggttccaattgacaagcttttgattttaacgacttttaacgacaacttgagaagatcaaaaaacaactaattattcgaaacgatgagattcccatctattttcactgctgttttgttcgctgcttcttctgctttggctgctccagttaacactactactgaggatgaaactgctcaaattccagctgaagctgttattggttactctgatttggagggtgacttcgatgttgctgttttgccattctctaactctactaacaatggtttgttgttcattaacactactattgcttctattgctgctaaggaggaaggtgtttctttggagaagagagaagctgaggctgctgatttcgacgccgtcttgaaattctggggtccagttgaggcagattatacgtcacatggtggtttggtcctgacaagattatttaaggaacaccctgaaacccagaaactctttcctaaatttactgggattgcccaagcagacatggccggaaacgctgccatttctgctcacggagccaccgttctaaaaaagttaggcgagcttctgaaagctaaaggtaatcatgctgcaattttgaaacccatggctaacagccatgcaactaagcacaagattccaatcaacaactttaagttgatctccgaaatcatagtgaaggttatgcaagagaaggctggaatggatgctggtggccagcaagcattgcgtaatgtgatggctgccgtaatagcggaccttgaagctaattacaaggagctaggtttcagtggatgagaattaattcgccttagacatgactgttcctcagttcaagttgggcacttacgagaagaccggtcttgctagattctaatcaagaggatgtcagaatgccatttgcctgagagatgcaggcttcatttttgatacttttttatttgtaacctatatagtataggattttttttgtcattttgtttcttctcgtacgagcttgctcctgatcagcctatctcgcagctgatgaatatcttgtggtaggggtttgggaaaatcattcgagtttgatgtttttcttggtatttcccactcctcttcagagtacagaagattaagtgagacgttcgtttgtgcaagcttatcgataagctttaatgcggtagtttatcacagttaaattgctaacgcagtcaggcaccgtgtatgaaatctaacaatgcgctcatcgtcatcctcggcaccgtcaccctggatgctgtaggcataggcttggttatgccggtactgccgggcctcttgcgggatatcgtccattccgacagcatcgccagtcactatggcgtgctgctagcgctatatgcgttgatgcaatttctatgcgcacccgttctcggagcactgtccgaccgctttggccgccgcccagtcctgctcgcttcgctacttggagccactatcgactacgcgatcatggcgaccacacccgtcctgtggatctatcgaatctaaatgtaagttaaaatctctaaataattaaataagtcccagtttctccatacgaaccttaacagcattgcggtgagcatctagaccttcaacagcagccagatccatcactgcttggccaatatgtttcagtccctcaggagttacgtcttgtgaagtgatgaacttctggaaggttgcagtgttaactccgctgtattgacgggcatatccgtacgttggcaaagtgtggttggtaccggaggagtaatctccacaactctctggagagtaggcaccaacaaacacagatccagcgtgttgtacttgatcaacataagaagaagcattctcgatttgcaggatcaagtgttcaggagcgtactgattggacatttccaaagcctgctcgtaggttgcaaccgatagggttgtagagtgtgcaatacacttgcgtacaatttcaacccttggcaactgcacagcttggttgtgaacagcatcttcaattctggcaagctccttgtctgtcatatcgacagccaacagaatcacctgggaatcaataccatgttcagcttgagacagaaggtctgaggcaacgaaatctggatcagcgtatttatcagcaataactagaacttcagaaggcccagcaggcatgtcaatactacacagggctgatgtgtcattttgaaccatcatcttggcagcagtaacgaactggtttcctggaccaaatattttgtcacacttaggaacagtttctgttccgtaagccatagcagctactgcctgggcgcctcctgctagcacgatacacttagcaccaaccttgtgggcaacgtagatgacttctggggtaagggtaccatccttcttaggtggagatgcaaaaacaatttctttgcaaccagcaactttggcaggaacacccagcatcagggaagtggaaggcagaattgcggttccaccaggaatatagaggccaactttctcaataggtcttgcaaaacgagagcagactacaccagggcaagtctcaacttgcaacgtctccgttagttgagcttcatggaatttcctgacgttatctatagagagatcaatggctctcttaacgttatctggcaattgcataagttcctctgggaaaggagcttctaacacaggtgtcttcaaagcgactccatcaaacttggcagttagttctaaaagggctttgtcaccattttgacgaacattgtcgacaattggtttgactaattccataatctgttccgttttctggataggacgacgaagggcatcttcaatttcttgtgaggaggccttagaaacgtcaattttgcacaattcaatacgaccttcagaagggacttctttaggtttggattcttctttaggttgttccttggtgtatcctggcttggcatctcctttccttctagtgacctttagggacttcatatccaggtttctctccacctcgtccaacgtcacaccgtacttggcacatctaactaatgcaaaataaaataagtcagcacattcccaggctatatcttccttggatttagcttctgcaagttcatcagcttcctccctaattttagcgttcaacaaaacttcgtcgtcaaataaccgtttggtataagaaccttctggagcattgctcttacgatcccacaaggtggcttccatggctctaagaccctttgattggccaaaacaggaagtgcgttccaagtgacagaaaccaacacctgtttgttcaaccacaaatttcaagcagtctccatcacaatccaattcgatacccagcaacttttgagttgctccagatgtagcacctttataccacaaaccgtgacgacgagattggtagactccagtttgtgtccttatagcctccggaatagactttttggacgagtacaccaggcccaacgagtaattagaagagtcagccaccaaagtagtgaatagaccatcggggcggtcagtagtcaaagacgccaacaaaatttcactgacagggaactttttgacatcttcagaaagttcgtattcagtagtcaattgccgagcatcaataatggggattataccagaagcaacagtggaagtcacatctaccaactttgcggtctcagaaaaagcataaacagttctactaccgccattagtgaaacttttcaaatcgcccagtggagaagaaaaaggcacagcgatactagcattagcgggcaaggatgcaactttatcaaccagggtcctatagataaccctagcgcctgggatcatcctttggacaactctttctgccaaatctaggtccaaaatcacttcattgataccattattgtacaacttgagcaagttgtcgatcagctcctcaaattggtcctctgtaacggatgactcaacttgcacattaacttgaagctcagtcgattgagtgaacttgatcaggttgtgcagctggtcagcagcatagggaaacacggcttttcctaccaaactcaaggaattatcaaactctgcaacacttgcgtatgcaggtagcaagggaaatgtcatacttgaagtcggacagtgagtgtagtcttgagaaattctgaagccgtatttttattatcagtgagtcagtcatcaggagatcctctacgccggacgcatcgtggccggcatcaccggcgccacaggtgcggttgctggcgcctatatcgccgacatcaccgatggggaagatcgggctcgccacttcgggctcatgagcgcttgtttcggcgtgggtatggtggcaggccccgtggccgggggactgttgggcgccatctccttgcatgcaccattccttgcggcggcggtgctcaacggcctcaacctactactgggctgcttcctaatgcaggagtcgcataagggagagcgtcgagtatctatgattggaagtatgggaatggtgatacccgcattcttcagtgtcttgaggtctcctatcagattatgcccaactaaagcaaccggaggaggagatttcatggtaaatttctctgacttttggtcatcagtagactcgaactgtgagactatctcggttatgacagcagaaatgtccttcttggagacagtaaatgaagtcccaccaataaagaaatccttgttatcaggaacaaacttcttgtttcgaactttttcggtgccttgaactataaaatgtagagtggatatgtcgggtaggaatggagcgggcaaatgcttaccttctggaccttcaagaggtatgtagggtttgtagatactgatgccaacttcagtgacaacgttgctatttcgttcaaaccattccgaatccagagaaatcaaagttgtttgtctactattgatccaagccagtgcggtcttgaaactgacaatagtgtgctcgtgttttgaggtcatctttgtatgaataaatctagtctttgatctaaataatcttgacgagccaaggcgataaatacccaaatctaaaactcttttaaaacgttaaaaggacaagtatgtctgcctgtattaaaccccaaatcagctcgtagtctgatcctcatcaacttgaggggcactatcttgttttagagaaatttgcggagatgcgatatcgagaaaaaggtacgctgattttaaacgtgaaatttatctcaagatct

SEQ ID NO: 28 - DNA, 6027 bp, synthetic construct
  source 1..6027: mol_type = other DNA; note = Nucleotide sequence of heterologous nucleic acid molecule comprising a nucleic acid sequence encoding a sword fish myoglobin
aacatccaaagacgaaaggttgaatgaaacctttttgccatccgacatccacaggtccattctcacacataagtgccaaacgcaacaggaggggatacactagcagcagaccgttgcaaacgcaggacctccactcctcttctcctcaacacccacttttgccatcgaaaaaccagcccagttattgggcttgattggagctcgctcattccaattccttctattaggctactaacaccatgactttattagcctgtctatcctggcccccctggcgaggttcatgtttgtttatttccgaatgcaacaagctccgcattacacccgaacatcactccagatgagggctttctgagtgtggggtcaaatagtttcatgttccccaaatggcccaaaactgacagtttaaacgctgtcttggaacctaatatgacaaaagcgtgatctcatccaagatgaactaagtttggttcgttgaaatgctaacggccagttggtcaaaaagaaacttccaaaagtcgccataccgtttgtcttgtttggtattgattgacgaatgctcaaaaataatctcattaatgcttagcgcagtctctctatcgcttctgaaccccggtgcacctgtgccgaaacgcaaatggggaaacacccgctttttggatgattatgcattgtctccacattgtatgcttccaagattctggtgggaatactgctgatagcctaacgttcatgatcaaaatttaactgttctaacccctacttgacagcaatatataaacagaaggaagctgccctgtcttaaacctttttttttatcatcattattagcttactttcataattgcgactggttccaattgacaagcttttgattttaacgacttttaacgacaacttgagaagatcaaaaaacaactaattattcgaaacgatgagattcccatctattttcactgctgttttgttcgctgcttcttctgctttggctgctccagttaacactactactgaggatgaaactgctcaaattccagctgaagctgttattggttactctgatttggagggtgacttcgatgttgctgttttgccattctctaactctactaacaatggtttgttgttcattaacactactattgcttctattgctgctaaggaggaaggtgtttctttggagaagagagaagctgaggctgccgaatttgaagtagttttaaagcattggggtcctgtggaggccgactatgcttcacatggcaacttagttctcacccgtctatttacagaacatccagacacacagaaactattccccaagttcgctggaatcgctcaaggggatatggccggtaacgctgcaatctccgctcacggtgcgaccgtcttgaaaaaattgggagagctgcttaaggctaagggaaatcacgccactaccctgaaagctttggcaactacgcatgcaacaaaacacaaaattccaatcaagaattttgaattgattgccgaagttataggtaaagtcatggaggaaaaggccggacttgattctgtgggtagggaggcattaagagatgtaatggcaagagttattgctgacattgatgctacttacaaggagttgggtttcactggctgagaattaattcgccttagacatgactgttcctcagttcaagttgggcacttacgagaagaccggtcttgctagattctaatcaagaggatgtcagaatgccatttgcctgagagatgcaggcttcatttttgatacttttttatttgtaacctatatagtataggattttttttgtcattttgtttcttctcgtacgagcttgctcctgatcagcctatctcgcagctgatgaatatcttgtggtaggggtttgggaaaatcattcgagtttgatgtttttcttggtatttcccactcctcttcagagtacagaagattaagtgagacgttcgtttgtgcaagcttatcgataagctttaatgcggtagtttatcacagttaaattgctaacgcagtcaggcaccgtgtatgaaatctaacaatgcgctcatcgtcatcctcggcaccgtcaccctggatgctgtaggcataggcttggttatgccggtactgccgggcctcttgcgggatatcgtccattccgacagcatcgccagtcactatggcgtgctgctagcgctatatgcgttgatgcaatttctatgcgcacccgttctcggagcactgtccgaccgctttggccgccgcccagtcctgctcgcttcgctacttggagccactatcgactacgcgatcatggcgaccacacccgtcctgtggatctatcgaatctaaatgtaagttaaaatctctaaataattaaataagtcccagtttctccatacgaaccttaacagcattgcggtgagcatctagaccttcaacagcagccagatccatcactgcttggccaatatgtttcagtccctcaggagttacgtcttgtgaagtgatgaacttctggaaggttgcagtgttaactccgctgtattgacgggcatatccgtacgttggcaaagtgtggttggtaccggaggagtaatctccacaactctctggagagtaggcaccaacaaacacagatccagcgtgttgtacttgatcaacataagaagaagcattctcgatttgcaggatcaagtgttcaggagcgtactgattggacatttccaaagcctgctcgtaggttgcaaccgatagggttgtagagtgtgcaatacacttgcgtacaatttcaacccttggcaactgcacagcttggttgtgaacagcatcttcaattctggcaagctccttgtctgtcatatcgacagccaacagaatcacctgggaatcaataccatgttcagcttgagacagaaggtctgaggcaacgaaatctggatcagcgtatttatcagcaataactagaacttcagaaggcccagcaggcatgtcaatactacacagggctgatgtgtcattttgaaccatcatcttggcagcagtaacgaactggtttcctggaccaaatattttgtcacacttaggaacagtttctgttccgtaagccatagcagctactgcctgggcgcctcctgctagcacgatacacttagcaccaaccttgtgggcaacgtagatgacttctggggtaagggtaccatccttcttaggtggagatgcaaaaacaatttctttgcaaccagcaactttggcaggaacacccagcatcagggaagtggaaggcagaattgcggttccaccaggaatatagaggccaactttctcaataggtcttgcaaaacgagagcagactacaccagggcaagtctcaacttgcaacgtctccgttagttgagcttcatggaatttcctgacgttatctatagagagatcaatggctctcttaacgttatctggcaattgcataagttcctctgggaaaggagcttctaacacaggtgtcttcaaagcgactccatcaaacttggcagttagttctaaaagggctttgtcaccattttgacgaacattgtcgacaattggtttgactaattccataatctgttccgttttctggataggacgacgaagggcatcttcaatttcttgtgaggaggccttagaaacgtcaattttgcacaattcaatacgaccttcagaagggacttctttaggtttggattcttctttaggttgttccttggtgtatcctggcttggcatctcctttccttctagtgacctttagggacttcatatccaggtttctctccacctcgtccaacgtcacaccgtacttggcacatctaactaatgcaaaataaaataagtcagcacattcccaggctatatcttccttggatttagcttctgcaagttcatcagcttcctccctaattttagcgttcaacaaaacttcgtcgtcaaataaccgtttggtataagaaccttctggagcattgctcttacgatcccacaaggtggcttccatggctctaagaccctttgattggccaaaacaggaagtgcgttccaagtgacagaaaccaacacctgtttgttcaaccacaaatttcaagcagtctccatcacaatccaattcgatacccagcaacttttgagttgctccagatgtagcacctttataccacaaaccgtgacgacgagattggtagactccagtttgtgtccttatagcctccggaatagactttttggacgagtacaccaggcccaacgagtaattagaagagtcagccaccaaagtagtgaatagaccatcggggcggtcagtagtcaaagacgccaacaaaatttcactgacagggaactttttgacatcttcagaaagttcgtattcagtagtcaattgccgagcatcaataatggggattataccagaagcaacagtggaagtcacatctaccaactttgcggtctcagaaaaagcataaacagttctactaccgccattagtgaaacttttcaaatcgcccagtggagaagaaaaaggcacagcgatactagcattagcgggcaaggatgcaactttatcaaccagggtcctatagataaccctagcgcctgggatcatcctttggacaactctttctgccaaatctaggtccaaaatcacttcattgataccattattgtacaacttgagcaagttgtcgatcagctcctcaaattggtcctctgtaacggatgactcaacttgcacattaacttgaagctcagtcgattgagtgaacttgatcaggttgtgcagctggtcagcagcatagggaaacacggcttttcctaccaaactcaaggaattatcaaactctgcaacacttgcgtatgcaggtagcaagggaaatgtcatacttgaagtcggacagtgagtgtagtcttgagaaattctgaagccgtatttttattatcagtgagtcagtcatcaggagatcctctacgccggacgcatcgtggccggcatcaccggcgccacaggtgcggttgctggcgcctatatcgccgacatcaccgatggggaagatcgggctcgccacttcgggctcatgagcgcttgtttcggcgtgggtatggtggcaggccccgtggccgggggactgttgggcgccatctccttgcatgcaccattccttgcggcggcggtgctcaacggcctcaacctactactgggctgcttcctaatgcaggagtcgcataagggagagcgtcgagtatctatgattggaagtatgggaatggtgatacccgcattcttcagtgtcttgaggtctcctatcagattatgcccaactaaagcaaccggaggaggagatttcatggtaaatttctctgacttttggtcatcagtagactcgaactgtgagactatctcggttatgacagcagaaatgtccttcttggagacagtaaatgaagtcccaccaataaagaaatccttgttatcaggaacaaacttcttgtttcgaactttttcggtgccttgaactataaaatgtagagtggatatgtcgggtaggaatggagcgggcaaatgcttaccttctggaccttcaagaggtatgtagggtttgtagatactgatgccaacttcagtgacaacgttgctatttcgttcaaaccattccgaatccagagaaatcaaagttgtttgtctactattgatccaagccagtgcggtcttgaaactgacaatagtgtgctcgtgttttgaggtcatctttgtatgaataaatctagtctttgatctaaataatcttgacgagccaaggcgataaatacccaaatctaaaactcttttaaaacgttaaaaggacaagtatgtctgcctgtattaaaccccaaatcagctcgtagtctgatcctcatcaacttgaggggcactatcttgttttagagaaatttgcggagatgcgatatcgagaaaaaggtacgctgattttaaacgtgaaatttatctcaagatct